European Patent Application EP 4 810 513 A1, published September 23, 2026. Title: SINGLE DOMAIN ANTIBODY SPECIFICALLY BINDING TO SOX2, FUSION PROTEIN COMPRISING THE SAME, AND USE THEREOF. Applicant: 주식회사 제넥신. The sequence listing filed with the application follows.

SEQUENCE LISTING (249 sequences)

SEQ ID NO: 1 - protein, 317 aa, synthetic construct
  REGION 1..317: note = huSOX2
MYNMMETELKPPGPQQTSGGGGGNSTAAAAGGNQKNSPDRVKRPMNAFMVWSRGQRRKMAQENPKMHNSEISKRLGAEWKLLSETEKRPFIDEAKRLRALHMKEHPDYKYRPRRKTKTLMKKDKYTLPGGLLAPGGNSMASGVGVGAGLGAGVNQRMDSYAHMNGWSNGSYSMMQDQLGYPQHPGLNAHGAAQMQPMHRYDVSALQYNSMTSSQTYMNGSPTYSMSYSQQGTPGMALGSMGSVVKSEASSSPPVVTSSSHSRAPCQAGDLRDMISMYLPGAEVPEPAAPSRLHMSQHYQSGPVPGTAINGTLPLSHM

SEQ ID NO: 2 - protein, 273 aa, synthetic construct
  REGION 1..273: note = cynoSOX2
MNAFMVWSRGQRRKMAQENPKMHNSEISKRLGAEWKLLSETEKRPFIDEAKRLRALHMKEHPDYKYRPRRKTKTLMKKDKYTLPGGLLAPGGNSMASGVGVGAGLGAGVNQRMDSYAHMNGWSNGSYSMMQDQLGYPQHPGLNAHGAAQMQPMHRYDVSALQYNSMTSSQTYMNGSPTYSMSYSQQGTPGMALGSMGSVVKSEASSSPPVVTSSSHSRAPCQAGDLRDMISMYLPGAEVPEPAAPSRLHMSQHYQSGPVPGTAINGTLPLSHM

SEQ ID NO: 3 - protein, 446 aa, synthetic construct
  REGION 1..446: note = huSOX3
MRPVRENSSGARSPRVPADLARSILISLPFPPDSLAHRPPSSAPTESQGLFTVAAPAPGAPSPPATLAHLLPAPAMYSLLETELKNPVGTPTQAAGTGGPAAPGGAGKSSANAAGGANSGGGSSGGASGGGGGTDQDRVKRPMNAFMVWSRGQRRKMALENPKMHNSEISKRLGADWKLLTDAEKRPFIDEAKRLRAVHMKEYPDYKYRPRRKTKTLLKKDKYSLPSGLLPPGAAAAAAAAAAAAAAASSPVGVGQRLDTYTHVNGWANGAYSLVQEQLGYAQPPSMSSPPPPPALPPMHRYDMAGLQYSPMMPPGAQSYMNVAAAAAAASGYGGMAPSATAAAAAAYGQQPATAAAAAAAAAAMSLGPMGSVVKSEPSSPPPAIASHSQRACLGDLRDMISMYLPPGGDAADAASPLPGGRLHGVHQHYQGAGTAVNGTVPLTHI

SEQ ID NO: 4 - protein, 184 aa, synthetic construct
  REGION 1..184: note = huSOX2 135-317
MGGNSMASGVGVGAGLGAGVNQRMDSYAHMNGWSNGSYSMMQDQLGYPQHPGLNAHGAAQMQPMHRYDVSALQYNSMTSSQTYMNGSPTYSMSYSQQGTPGMALGSMGSVVKSEASSSPPVVTSSSHSRAPCQAGDLRDMISMYLPGAEVPEPAAPSRLHMSQHYQSGPVPGTAINGTLPLSHM

SEQ ID NO: 5 - protein, 118 aa, synthetic construct
  REGION 1..118: note = S14
QVKLEESGGGSVQTGGSLRLTCAASGSIFSMNRMGWFRQAPGKERELVAVIDSKRNKTHYADSVKGRFTISRDNAKNTVDLQMNSLKPEDTAIYYCTAWTGRPPRGYWGQGTQVTVSS

SEQ ID NO: 6 - protein, 115 aa, synthetic construct
  REGION 1..115: note = 1A5
EVQLVESGGGLVQPGGSLRLSCAASGSTYTTYSMGWFRQAPGKEREFVGAIHWSGGRTYYADSVKGRFTISADNSKNTAYLQMNSLKPEDTAVYYCASRVDDRVWGQGTLVTVSS

SEQ ID NO: 7 - protein, 115 aa, synthetic construct
  REGION 1..115: note = 1A9
EVQLVESGGGLVQPGGSLRLSCAASGRTFSTYSMGWFRQAPGKEREFVAAIRWTAGTTYYADSVKGRFTISADNSKNTAYLQMNSLKPEDTAVYYCASRVDDRVWGQGTLVTVSS

SEQ ID NO: 8 - protein, 115 aa, synthetic construct
  REGION 1..115: note = 1A11
EVQLVESGGGLVQPGGSLRLSCAASGSTYTTYSMGWFRQAPGKEREFVAAIHWSGGGTYYADSVKGRFTISADNSKNTAYLQMNSLKPEDTAVYYCASRVDDRVWGQGTLVTVSS

SEQ ID NO: 9 - protein, 116 aa, synthetic construct
  REGION 1..116: note = 1B9
EVQLVESGGGLVQPGGSLRLSCAASGLTFSTYSMGWFRQAPGKEREFVAAITWNSGRRTYYADSVKGRFTISADNSKNTAYLQMNSLKPEDTAVYYCASRVDDRVWGQGTLVTVSS

SEQ ID NO: 10 - protein, 115 aa, synthetic construct
  REGION 1..115: note = 1C2
EVQLVESGGGLVQPGGSLRLSCAASGSTYTTYSMGWFRQAPGKEREFVAAIRWSGGTTYYADSVKGRFTISADNSKNTAYLQMNSLKPEDTAVYYCASRVDDRVWGQGTLVTVSS

SEQ ID NO: 11 - protein, 115 aa, synthetic construct
  REGION 1..115: note = 1C11
EVQLVESGGGLVQPGGSLRLSCAASGSTYTTYSMGWFRQAPGKEREFVGAIRWSGGTTYYADSVKGRFTISADNSKNTAYLQMNSLKPEDTAVYYCASRVDDRVWGQGTLVTVSS

SEQ ID NO: 12 - protein, 115 aa, synthetic construct
  REGION 1..115: note = 1C12
EVQLVESGGGLVQPGGSLRLSCAASGSTYTTYSMGWFRQAPGKEREFVAAIRWSGGSTHYADSVKGRFTISADNSKNTAYLQMNSLKPEDTAVYYCASRVDDRVWGQGTLVTVSS

SEQ ID NO: 13 - protein, 119 aa, synthetic construct
  REGION 1..119: note = 1C4
EVQLVESGGGLVQPGGSLRLSCAASGGGFRGNAVMGWFRQAPGKERELVAAIRGSGEDTYYADSVKGRFTISADNSKNTAYLQMNSLKPEDTAVYYCAGGWRRGYFQDWGQGTLVTVSS

SEQ ID NO: 14 - protein, 118 aa, synthetic construct
  REGION 1..118: note = 2E8
EVQLVESGGGLVQPGGSLRLSCAASGFTLDYYGMGWFRQAPGKEREFVAAISRSGGSTVYADSVKGRFTISADNSKNTAYLQMNSLKPEDTAVYYCAREVVRGGINYWGQGTLVTVSS

SEQ ID NO: 15 - protein, 126 aa, synthetic construct
  REGION 1..126: note = 3F11
DVQLVESGGGLVQPGGSLRLSCATSGFTFSSSTMSWVRQVPGAGPEWVAVDNPGGKKNYIDSVAGRFTIARDNDANSLSLVMNGLRPEDTARYFCARVLSFKIYEGDKWALEWDYRGPGTQVTVSS

SEQ ID NO: 16 - protein, 126 aa, synthetic construct
  REGION 1..126: note = 3A2
EVQLVESGGEQVQPGSSLKLSCSVSGLMISGHAMSWVRQVPGAGPEWVAVDNPGGKKNYIDSVAGRFTIARDNDANSLSLVMNGLRPEDTARYFCARVLSFKIYEGDKWALEWDYRGPGTQVTVSS

SEQ ID NO: 17 - protein, 126 aa, synthetic construct
  REGION 1..126: note = 3H9
QVQLVESGGEQVQPGSSLKLSCSVSGLMISGHAMSWVRQVPGAGPEWVAVDNPGGKKNYIDSVAGRFTIARDNDANSLSLVMNGLRPEDTARYFCARVLSFKIYGGDKWALEWDYRGPGTQVTVSS

SEQ ID NO: 18 - protein, 262 aa, synthetic construct
  REGION 1..262: note = bTrCP190-228
DPAEAVLQEKALKFMNSSEREDCNNGEPPRKIIPEKNSLRQTYNSCARLCLNQETVCLASTAMKTENCVAKTKLANGTSSMIVPKQRKLSASYEKEKELCVKYFEQWSESDQVEFVEHLISQMCHYQHGHINSYLKPMLQRDFITALPARGLDHIAENILSYLDAKSLCAAELVCKEWYRVTSDGMLWKKLIERMVRTDSLWRGLAERRGWGQYLFKNKPPDGNAPPNSFYRALYPKIIQDIETIESNWRCGRHSLQRIHCR

SEQ ID NO: 19 - protein, 175 aa, synthetic construct
  REGION 1..175: note = SKP22-176
HRKHLQEIPDLSSNVATSFTWGWDSSKTSELLSGMGVSALEKEEPDSENIPQELLSNLGHPESPPRKRLKSKGSDKDFVIVRRPKLNRENFPGVSWDSLPDELLLGIFSCLCLPELLKVSGVCKRWYRLASDESLWQTLDLTGKNLHPDVTGRLLSQGVIAFRCPRSFMDQPLAE

SEQ ID NO: 20 - protein, 62 aa, synthetic construct
  REGION 1..62: note = VHL152-213
TLPVYTLKERCLQVVRSLVKPENYRRLDIVRSLYEDLEDHPNVQKDLERLTQERIAHQRMGD

SEQ ID NO: 21 - protein, 208 aa, synthetic construct
  REGION 1..208: note = SPOP167-374
SVNISGQNTMNMVKVPECRLADELGGLWENSRFTDCCLCVAGQEFQAHKAILAARSPVFSAMFEHEMEESKKNRVEINDVEPEVFKEMMCFIYTGKAPNLDKMADDLLAAADKYALERLKVMCEDALCSNLSVENAAEILILADLHSADQLKTQAVDFINYHASDVLETSGWKSMVVSHPHLVAEAYRSLASAQCPFLGPPRKRLKQS

SEQ ID NO: 22 - protein, 56 aa, synthetic construct
  REGION 1..56: note = SOCS2143-198
PRNGTVHLYLTKPLYTSAPSLQHLCRLTINKCTGAIWGLPLPTRLKDYLEEYKFQV

SEQ ID NO: 23 - protein, 176 aa, synthetic construct
  REGION 1..176: note = CHIP128-303
RLNFGDDIPSALRIAKKKRWNSIEERRIHQESELHSYLSRLIAAERERELEECQRNHEGDEDDSHVRAQQACIEAKHDKYMADMDELFSQVDEKRKKRDIPDYLCGKISFELMREPCITPSGITYDRKDIEEHLQRVGHFDPVTRSPLTQEQLIPNLAMKEVIDAFISENGWVEDY

SEQ ID NO: 24 - protein, 113 aa, synthetic construct
  REGION 1..113: note = DDB2 2-114
APKKRPETQKTSEIVLRPRNKRSRSPLELEPEAKKLCAKGSGPSRRCDSDCLWVGLAGPQILPPCRSIVRTLHQHKLGRASWPSVQQGLQQSFLHTLDSYRILQKAAPFDRRA

SEQ ID NO: 25 - protein, 319 aa, synthetic construct
  REGION 1..319: note = CRBN2-320
AGEGDQQDAAHNMGNHLPLLPAESEEEDEMEVEDQDSKEAKKPNIINFDTSLPTSHTYLGADMEEFHGRTLHDDDSCQVIPVLPQVMMILIPGQTLPLQLFHPQEVSMVRNLIQKDRTFAVLAYSNVQEREAQFGTTAEIYAYREEQDFGIEIVKVKAIGRQRFKVLELRTQSDGIQQAKVQILPECVLPSTMSAVQLESLNKCQIFPSKPVSREDQCSYKWWQKYQKRKFHCANLTSWPRWLYSLYDAETLMDRIKKQLREWDENLKDDSLPSNPIDFSYRVAACLPIDDVLRIQLLKIGSAIQRLRCELDIMNKCTS

SEQ ID NO: 26 - protein, 70 aa, synthetic construct
  REGION 1..70: note = ASB1 266-335
VKWESLGPESRGRRKVDPEALQVFKEARSVPRTLLCLCRVAVRRALGKHRLHLIPSLPLPDPIKKFLLHE

SEQ ID NO: 27 - protein, 84 aa, synthetic construct
  REGION 1..84: note = TRIM21 2-85
ASAARLTMMWEEVTCPICLDPFVEPVSIECGHSFCQECISQVGKGGGSVCPVCRQRFLLKNLRPNRQLANMVNNLKEISQEARE

SEQ ID NO: 28 - protein, 120 aa, synthetic construct
  REGION 1..120: note = RNF4 71-190
DERRRPRRNARRLPQDHADSCVVSSDDEELSRDRDVYVTTHTPRNARDEGATGLRPSGTVSCPICMDGYSEIVQNGRLIVSTECGHVFCSQCLRDSLKNANTCPTCRKKINHKRYHPIYI

SEQ ID NO: 29 - protein, 146 aa, synthetic construct
  REGION 1..146: note = UBE2D1 2-147
ALKRIQKELSDLQRDPPAHCSAGPVGDDLFHWQATIMGPPDSAYQGGVFFLTVHFPTDYPFKPPKIAFTTKIYHPNINSNGSICLDILRSQWSPALTVSKVLLSICSLLCDPNPDDPLVPDIAQIYKSDKEKYNRHAREWTQKYAM

SEQ ID NO: 30 - protein, 146 aa, synthetic construct
  REGION 1..146: note = UBE2D4 2-147
ALKRIQKELTDLQRDPPAQCSAGPVGDDLFHWQATIMGPNDSPYQGGVFFLTIHFPTDYPFKPPKVAFTTKIYHPNINSNGSICLDILRSQWSPALTVSKVLLSICSLLCDPNPDDPLVPEIAHTYKADREKYNRLAREWTQKYAM

SEQ ID NO: 31 - protein, 90 aa, synthetic construct
  REGION 1..90: note = ZNFR1 138-227
SSHSGFKCPICSKSVASDEMEMHFIMCLSKPRLSYNDDVLTKDAGECVICLEELLQGDTIARLPCLCIYHKSCIDSWFEVNRSCPEHPAD

SEQ ID NO: 32 - protein, 333 aa, synthetic construct
  REGION 1..333: note = huSOX2.Myc
MYNMMETELKPPGPQQTSGGGGGNSTAAAAGGNQKNSPDRVKRPMNAFMVWSRGQRRKMAQENPKMHNSEISKRLGAEWKLLSETEKRPFIDEAKRLRALHMKEHPDYKYRPRRKTKTLMKKDKYTLPGGLLAPGGNSMASGVGVGAGLGAGVNQRMDSYAHMNGWSNGSYSMMQDQLGYPQHPGLNAHGAAQMQPMHRYDVSALQYNSMTSSQTYMNGSPTYSMSYSQQGTPGMALGSMGSVVKSEASSSPPVVTSSSHSRAPCQAGDLRDMISMYLPGAEVPEPAAPSRLHMSQHYQSGPVPGTAINGTLPLSHMTRTRPLEQKLISEEDL

SEQ ID NO: 33 - protein, 392 aa, synthetic construct
  REGION 1..392: note = Flag tag-bTrCP190-228.GS.S14
DYKDDDDKTRDPAEAVLQEKALKFMNSSEREDCNNGEPPRKIIPEKNSLRQTYNSCARLCLNQETVCLASTAMKTENCVAKTKLANGTSSMIVPKQRKLSASYEKEKELCVKYFEQWSESDQVEFVEHLISQMCHYQHGHINSYLKPMLQRDFITALPARGLDHIAENILSYLDAKSLCAAELVCKEWYRVTSDGMLWKKLIERMVRTDSLWRGLAERRGWGQYLFKNKPPDGNAPPNSFYRALYPKIIQDIETIESNWRCGRHSLQRIHCRGSQVKLEESGGGSVQTGGSLRLTCAASGSIFSMNRMGWFRQAPGKERELVAVIDSKRNKTHYADSVKGRFTISRDNAKNTVDLQMNSLKPEDTAIYYCTAWTGRPPRGYWGQGTQVTVSS

SEQ ID NO: 34 - protein, 305 aa, synthetic construct
  REGION 1..305: note = Flag tag-SKP22-176.GS.S14
DYKDDDDKTRHRKHLQEIPDLSSNVATSFTWGWDSSKTSELLSGMGVSALEKEEPDSENIPQELLSNLGHPESPPRKRLKSKGSDKDFVIVRRPKLNRENFPGVSWDSLPDELLLGIFSCLCLPELLKVSGVCKRWYRLASDESLWQTLDLTGKNLHPDVTGRLLSQGVIAFRCPRSFMDQPLAEGSQVKLEESGGGSVQTGGSLRLTCAASGSIFSMNRMGWFRQAPGKERELVAVIDSKRNKTHYADSVKGRFTISRDNAKNTVDLQMNSLKPEDTAIYYCTAWTGRPPRGYWGQGTQVTVSS

SEQ ID NO: 35 - protein, 192 aa, synthetic construct
  REGION 1..192: note = Flag tag-S14.GS.VHL152-213
DYKDDDDKTRQVKLEESGGGSVQTGGSLRLTCAASGSIFSMNRMGWFRQAPGKERELVAVIDSKRNKTHYADSVKGRFTISRDNAKNTVDLQMNSLKPEDTAIYYCTAWTGRPPRGYWGQGTQVTVSSGSTLPVYTLKERCLQVVRSLVKPENYRRLDIVRSLYEDLEDHPNVQKDLERLTQERIAHQRMGD

SEQ ID NO: 36 - protein, 338 aa, synthetic construct
  REGION 1..338: note = Flag tag-S14.GS.SPOP167-374
DYKDDDDKTRQVKLEESGGGSVQTGGSLRLTCAASGSIFSMNRMGWFRQAPGKERELVAVIDSKRNKTHYADSVKGRFTISRDNAKNTVDLQMNSLKPEDTAIYYCTAWTGRPPRGYWGQGTQVTVSSGSSVNISGQNTMNMVKVPECRLADELGGLWENSRFTDCCLCVAGQEFQAHKAILAARSPVFSAMFEHEMEESKKNRVEINDVEPEVFKEMMCFIYTGKAPNLDKMADDLLAAADKYALERLKVMCEDALCSNLSVENAAEILILADLHSADQLKTQAVDFINYHASDVLETSGWKSMVVSHPHLVAEAYRSLASAQCPFLGPPRKRLKQS

SEQ ID NO: 37 - protein, 186 aa, synthetic construct
  REGION 1..186: note = Flag tag-S14.GS.SOCS2 143-198
DYKDDDDKTRQVKLEESGGGSVQTGGSLRLTCAASGSIFSMNRMGWFRQAPGKERELVAVIDSKRNKTHYADSVKGRFTISRDNAKNTVDLQMNSLKPEDTAIYYCTAWTGRPPRGYWGQGTQVTVSSGSPRNGTVHLYLTKPLYTSAPSLQHLCRLTINKCTGAIWGLPLPTRLKDYLEEYKFQV

SEQ ID NO: 38 - protein, 306 aa, synthetic construct
  REGION 1..306: note = Flag tag-S14.GS.CHIP128-303
DYKDDDDKTRQVKLEESGGGSVQTGGSLRLTCAASGSIFSMNRMGWFRQAPGKERELVAVIDSKRNKTHYADSVKGRFTISRDNAKNTVDLQMNSLKPEDTAIYYCTAWTGRPPRGYWGQGTQVTVSSGSRLNFGDDIPSALRIAKKKRWNSIEERRIHQESELHSYLSRLIAAERERELEECQRNHEGDEDDSHVRAQQACIEAKHDKYMADMDELFSQVDEKRKKRDIPDYLCGKISFELMREPCITPSGITYDRKDIEEHLQRVGHFDPVTRSPLTQEQLIPNLAMKEVIDAFISENGWVEDY

SEQ ID NO: 39 - protein, 243 aa, synthetic construct
  REGION 1..243: note = Flag tag-DDB22-114.GS.S14
DYKDDDDKTRAPKKRPETQKTSEIVLRPRNKRSRSPLELEPEAKKLCAKGSGPSRRCDSDCLWVGLAGPQILPPCRSIVRTLHQHKLGRASWPSVQQGLQQSFLHTLDSYRILQKAAPFDRRAGSQVKLEESGGGSVQTGGSLRLTCAASGSIFSMNRMGWFRQAPGKERELVAVIDSKRNKTHYADSVKGRFTISRDNAKNTVDLQMNSLKPEDTAIYYCTAWTGRPPRGYWGQGTQVTVSS

SEQ ID NO: 40 - protein, 449 aa, synthetic construct
  REGION 1..449: note = Flag tag-CRBN2-320.GS.S14
DYKDDDDKTRAGEGDQQDAAHNMGNHLPLLPAESEEEDEMEVEDQDSKEAKKPNIINFDTSLPTSHTYLGADMEEFHGRTLHDDDSCQVIPVLPQVMMILIPGQTLPLQLFHPQEVSMVRNLIQKDRTFAVLAYSNVQEREAQFGTTAEIYAYREEQDFGIEIVKVKAIGRQRFKVLELRTQSDGIQQAKVQILPECVLPSTMSAVQLESLNKCQIFPSKPVSREDQCSYKWWQKYQKRKFHCANLTSWPRWLYSLYDAETLMDRIKKQLREWDENLKDDSLPSNPIDFSYRVAACLPIDDVLRIQLLKIGSAIQRLRCELDIMNKCTSGSQVKLEESGGGSVQTGGSLRLTCAASGSIFSMNRMGWFRQAPGKERELVAVIDSKRNKTHYADSVKGRFTISRDNAKNTVDLQMNSLKPEDTAIYYCTAWTGRPPRGYWGQGTQVTVSS

SEQ ID NO: 41 - protein, 200 aa, synthetic construct
  REGION 1..200: note = Flag tag-S14.GS.ASB1 266-335
DYKDDDDKTRQVKLEESGGGSVQTGGSLRLTCAASGSIFSMNRMGWFRQAPGKERELVAVIDSKRNKTHYADSVKGRFTISRDNAKNTVDLQMNSLKPEDTAIYYCTAWTGRPPRGYWGQGTQVTVSSGSVKWESLGPESRGRRKVDPEALQVFKEARSVPRTLLCLCRVAVRRALGKHRLHLIPSLPLPDPIKKFLLHE

SEQ ID NO: 42 - protein, 214 aa, synthetic construct
  REGION 1..214: note = Flag tag-TRIM212-85.GS.S14
DYKDDDDKTRASAARLTMMWEEVTCPICLDPFVEPVSIECGHSFCQECISQVGKGGGSVCPVCRQRFLLKNLRPNRQLANMVNNLKEISQEAREGSQVKLEESGGGSVQTGGSLRLTCAASGSIFSMNRMGWFRQAPGKERELVAVIDSKRNKTHYADSVKGRFTISRDNAKNTVDLQMNSLKPEDTAIYYCTAWTGRPPRGYWGQGTQVTVSS

SEQ ID NO: 43 - protein, 250 aa, synthetic construct
  REGION 1..250: note = Flag tag-S14.GS.RNF4 71-190
DYKDDDDKTRQVKLEESGGGSVQTGGSLRLTCAASGSIFSMNRMGWFRQAPGKERELVAVIDSKRNKTHYADSVKGRFTISRDNAKNTVDLQMNSLKPEDTAIYYCTAWTGRPPRGYWGQGTQVTVSSGSDERRRPRRNARRLPQDHADSCVVSSDDEELSRDRDVYVTTHTPRNARDEGATGLRPSGTVSCPICMDGYSEIVQNGRLIVSTECGHVFCSQCLRDSLKNANTCPTCRKKINHKRYHPIYI

SEQ ID NO: 44 - protein, 200 aa, synthetic construct
  REGION 1..200: note = Flag tag-3A2.GS.VHL152-213
DYKDDDDKTREVQLVESGGEQVQPGSSLKLSCSVSGLMISGHAMSWVRQVPGAGPEWVAVDNPGGKKNYIDSVAGRFTIARDNDANSLSLVMNGLRPEDTARYFCARVLSFKIYEGDKWALEWDYRGPGTQVTVSSGSTLPVYTLKERCLQVVRSLVKPENYRRLDIVRSLYEDLEDHPNVQKDLERLTQERIAHQRMGD

SEQ ID NO: 45 - protein, 346 aa, synthetic construct
  REGION 1..346: note = Flag tag-3A2.GS.SPOP167-374
DYKDDDDKTREVQLVESGGEQVQPGSSLKLSCSVSGLMISGHAMSWVRQVPGAGPEWVAVDNPGGKKNYIDSVAGRFTIARDNDANSLSLVMNGLRPEDTARYFCARVLSFKIYEGDKWALEWDYRGPGTQVTVSSGSSVNISGQNTMNMVKVPECRLADELGGLWENSRFTDCCLCVAGQEFQAHKAILAARSPVFSAMFEHEMEESKKNRVEINDVEPEVFKEMMCFIYTGKAPNLDKMADDLLAAADKYALERLKVMCEDALCSNLSVENAAEILILADLHSADQLKTQAVDFINYHASDVLETSGWKSMVVSHPHLVAEAYRSLASAQCPFLGPPRKRLKQS

SEQ ID NO: 46 - protein, 194 aa, synthetic construct
  REGION 1..194: note = Flag tag-3A2.GS.SOCS2 143-198
DYKDDDDKTREVQLVESGGEQVQPGSSLKLSCSVSGLMISGHAMSWVRQVPGAGPEWVAVDNPGGKKNYIDSVAGRFTIARDNDANSLSLVMNGLRPEDTARYFCARVLSFKIYEGDKWALEWDYRGPGTQVTVSSGSPRNGTVHLYLTKPLYTSAPSLQHLCRLTINKCTGAIWGLPLPTRLKDYLEEYKFQV

SEQ ID NO: 47 - protein, 314 aa, synthetic construct
  REGION 1..314: note = Flag tag-3A2.GS.CHIP128-303
DYKDDDDKTREVQLVESGGEQVQPGSSLKLSCSVSGLMISGHAMSWVRQVPGAGPEWVAVDNPGGKKNYIDSVAGRFTIARDNDANSLSLVMNGLRPEDTARYFCARVLSFKIYEGDKWALEWDYRGPGTQVTVSSGSRLNFGDDIPSALRIAKKKRWNSIEERRIHQESELHSYLSRLIAAERERELEECQRNHEGDEDDSHVRAQQACIEAKHDKYMADMDELFSQVDEKRKKRDIPDYLCGKISFELMREPCITPSGITYDRKDIEEHLQRVGHFDPVTRSPLTQEQLIPNLAMKEVIDAFISENGWVEDY

SEQ ID NO: 48 - protein, 208 aa, synthetic construct
  REGION 1..208: note = Flag tag-3A2GS.ASB1 266-335
DYKDDDDKTREVQLVESGGEQVQPGSSLKLSCSVSGLMISGHAMSWVRQVPGAGPEWVAVDNPGGKKNYIDSVAGRFTIARDNDANSLSLVMNGLRPEDTARYFCARVLSFKIYEGDKWALEWDYRGPGTQVTVSSGSVKWESLGPESRGRRKVDPEALQVFKEARSVPRTLLCLCRVAVRRALGKHRLHLIPSLPLPDPIKKFLLHE

SEQ ID NO: 49 - protein, 222 aa, unidentified
  REGION 1..222: note = Flag tag-TRIM21 2-85.GS.3A2
DYKDDDDKTRASAARLTMMWEEVTCPICLDPFVEPVSIECGHSFCQECISQVGKGGGSVCPVCRQRFLLKNLRPNRQLANMVNNLKEISQEAREGSEVQLVESGGEQVQPGSSLKLSCSVSGLMISGHAMSWVRQVPGAGPEWVAVDNPGGKKNYIDSVAGRFTIARDNDANSLSLVMNGLRPEDTARYFCARVLSFKIYEGDKWALEWDYRGPGTQVTVSS

SEQ ID NO: 50 - protein, 258 aa, synthetic construct
  REGION 1..258: note = Flag tag-3A2.GS.RNF4 71-190
DYKDDDDKTREVQLVESGGEQVQPGSSLKLSCSVSGLMISGHAMSWVRQVPGAGPEWVAVDNPGGKKNYIDSVAGRFTIARDNDANSLSLVMNGLRPEDTARYFCARVLSFKIYEGDKWALEWDYRGPGTQVTVSSGSDERRRPRRNARRLPQDHADSCVVSSDDEELSRDRDVYVTTHTPRNARDEGATGLRPSGTVSCPICMDGYSEIVQNGRLIVSTECGHVFCSQCLRDSLKNANTCPTCRKKINHKRYHPIYI

SEQ ID NO: 51 - protein, 284 aa, synthetic construct
  REGION 1..284: note = Flag tag-3A2.GS.UBE2D1 2-147
DYKDDDDKTREVQLVESGGEQVQPGSSLKLSCSVSGLMISGHAMSWVRQVPGAGPEWVAVDNPGGKKNYIDSVAGRFTIARDNDANSLSLVMNGLRPEDTARYFCARVLSFKIYEGDKWALEWDYRGPGTQVTVSSGSALKRIQKELSDLQRDPPAHCSAGPVGDDLFHWQATIMGPPDSAYQGGVFFLTVHFPTDYPFKPPKIAFTTKIYHPNINSNGSICLDILRSQWSPALTVSKVLLSICSLLCDPNPDDPLVPDIAQIYKSDKEKYNRHAREWTQKYAM

SEQ ID NO: 52 - protein, 284 aa, synthetic construct
  REGION 1..284: note = Flag tag-3A2.GS.UBE2D4 2-147
DYKDDDDKTREVQLVESGGEQVQPGSSLKLSCSVSGLMISGHAMSWVRQVPGAGPEWVAVDNPGGKKNYIDSVAGRFTIARDNDANSLSLVMNGLRPEDTARYFCARVLSFKIYEGDKWALEWDYRGPGTQVTVSSGSALKRIQKELTDLQRDPPAQCSAGPVGDDLFHWQATIMGPNDSPYQGGVFFLTIHFPTDYPFKPPKVAFTTKIYHPNINSNGSICLDILRSQWSPALTVSKVLLSICSLLCDPNPDDPLVPEIAHTYKADREKYNRLAREWTQKYAM

SEQ ID NO: 53 - protein, 228 aa, synthetic construct
  REGION 1..228: note = Flag tag-3A2.GS.ZNFR1 138-227
DYKDDDDKTREVQLVESGGEQVQPGSSLKLSCSVSGLMISGHAMSWVRQVPGAGPEWVAVDNPGGKKNYIDSVAGRFTIARDNDANSLSLVMNGLRPEDTARYFCARVLSFKIYEGDKWALEWDYRGPGTQVTVSSGSSSHSGFKCPICSKSVASDEMEMHFIMCLSKPRLSYNDDVLTKDAGECVICLEELLQGDTIARLPCLCIYHKSCIDSWFEVNRSCPEHPAD

SEQ ID NO: 54 - protein, 337 aa, synthetic construct
  REGION 1..337: note = huSOX2.V5
MYNMMETELKPPGPQQTSGGGGGNSTAAAAGGNQKNSPDRVKRPMNAFMVWSRGQRRKMAQENPKMHNSEISKRLGAEWKLLSETEKRPFIDEAKRLRALHMKEHPDYKYRPRRKTKTLMKKDKYTLPGGLLAPGGNSMASGVGVGAGLGAGVNQRMDSYAHMNGWSNGSYSMMQDQLGYPQHPGLNAHGAAQMQPMHRYDVSALQYNSMTSSQTYMNGSPTYSMSYSQQGTPGMALGSMGSVVKSEASSSPPVVTSSSHSRAPCQAGDLRDMISMYLPGAEVPEPAAPSRLHMSQHYQSGPVPGTAINGTLPLSHMTRTRPLGKPIPNPLLGLDST

SEQ ID NO: 55 - protein, 25 aa, synthetic construct
  REGION 1..25: note = FR1
QVKLEESGGGSVQTGGSLRLTCAAS

SEQ ID NO: 56 - protein, 8 aa, synthetic construct
  REGION 1..8: note = HCDR1
GSIFSMNR

SEQ ID NO: 57 - protein, 17 aa, synthetic construct
  REGION 1..17: note = FR2
MGWFRQAPGKERELVAV

SEQ ID NO: 58 - protein, 8 aa, synthetic construct
  REGION 1..8: note = HCDR2
IDSKRNKT

SEQ ID NO: 59 - protein, 38 aa, synthetic construct
  REGION 1..38: note = FR3
HYADSVKGRFTISRDNAKNTVDLQMNSLKPEDTAIYYC

SEQ ID NO: 60 - protein, 11 aa, synthetic construct
  REGION 1..11: note = HCDR3
TAWTGRPPRGY

SEQ ID NO: 61 - protein, 11 aa, synthetic construct
  REGION 1..11: note = FR4
WGQGTQVTVSS

SEQ ID NO: 62 - protein, 25 aa, synthetic construct [sequence omitted]

SEQ ID NO: 63 - protein, 8 aa, synthetic construct
  REGION 1..8: note = HCDR1
GSTYTTYS

SEQ ID NO: 64 - protein, 17 aa, synthetic construct
  REGION 1..17: note = FR2
MGWFRQAPGKEREFVGA

SEQ ID NO: 65 - protein, 8 aa, synthetic construct
  REGION 1..8: note = HCDR2
IHWSGGRT

SEQ ID NO: 66 - protein, 38 aa, synthetic construct
  REGION 1..38: note = FR3
YYADSVKGRFTISADNSKNTAYLQMNSLKPEDTAVYYC

SEQ ID NO: 67 - protein, 8 aa, synthetic construct
  REGION 1..8: note = HCDR3
ASRVDDRV

SEQ ID NO: 68 - protein, 11 aa, synthetic construct
  REGION 1..11: note = FR4
WGQGTLVTVSS

SEQ ID NO: 69 - protein, 8 aa, synthetic construct
  REGION 1..8: note = HCDR1
GRTFSTYS

SEQ ID NO: 70 - protein, 17 aa, synthetic construct
  REGION 1..17: note = FR2
MGWFRQAPGKEREFVAA

SEQ ID NO: 71 - protein, 8 aa, synthetic construct
  REGION 1..8: note = HCDR2
IRWTAGTT

SEQ ID NO: 72 - protein, 8 aa, synthetic construct
  REGION 1..8: note = HCDR2
IHWSGGGT

SEQ ID NO: 73 - protein, 8 aa, synthetic construct
  REGION 1..8: note = HCDR1
GLTFSTYS

SEQ ID NO: 74 - protein, 9 aa, synthetic construct
  REGION 1..9: note = HCDR2
ITWNSGRRT

SEQ ID NO: 75 - protein, 8 aa, synthetic construct
  REGION 1..8: note = HCDR2
IRWSGGTT

SEQ ID NO: 76 - protein, 8 aa, synthetic construct
  REGION 1..8: note = HCDR2
IRWSGGST

SEQ ID NO: 77 - protein, 38 aa, synthetic construct
  REGION 1..38: note = FR3
HYADSVKGRFTISADNSKNTAYLQMNSLKPEDTAVYYC

SEQ ID NO: 78 - protein, 8 aa, synthetic construct
  REGION 1..8: note = HCDR1
GFTLDYYG

SEQ ID NO: 79 - protein, 8 aa, synthetic construct
  REGION 1..8: note = HCDR2
ISRSGGST

SEQ ID NO: 80 - protein, 38 aa, synthetic construct
  REGION 1..38: note = FR3
VYADSVKGRFTISADNSKNTAYLQMNSLKPEDTAVYYC

SEQ ID NO: 81 - protein, 11 aa, synthetic construct
  REGION 1..11: note = HCDR3
AREVVRGGINY

SEQ ID NO: 82 - protein, 9 aa, synthetic construct
  REGION 1..9: note = HCDR1
GGGFRGNAV

SEQ ID NO: 83 - protein, 17 aa, synthetic construct
  REGION 1..17: note = FR2
MGWFRQAPGKERELVAA

SEQ ID NO: 84 - protein, 8 aa, synthetic construct
  REGION 1..8: note = HCDR2
IRGSGEDT

SEQ ID NO: 85 - protein, 11 aa, synthetic construct
  REGION 1..11: note = HCDR3
AGGWRRGYFQD

SEQ ID NO: 86 - protein, 25 aa, synthetic construct
  REGION 1..25: note = FR1
DVQLVESGGGLVQPGGSLRLSCATS

SEQ ID NO: 87 - protein, 8 aa, synthetic construct
  REGION 1..8: note = HCDR1
GFTFSSST

SEQ ID NO: 88 - protein, 17 aa, synthetic construct
  REGION 1..17: note = FR2
MSWVRQVPGAGPEWVAV

SEQ ID NO: 89 - protein, 7 aa, synthetic construct
  REGION 1..7: note = HCDR2
DNPGGKK

SEQ ID NO: 90 - protein, 38 aa, synthetic construct
  REGION 1..38: note = FR3
NYIDSVAGRFTIARDNDANSLSLVMNGLRPEDTARYFC

SEQ ID NO: 91 - protein, 20 aa, synthetic construct
  REGION 1..20: note = HCDR3
ARVLSFKIYEGDKWALEWDY

SEQ ID NO: 92 - protein, 11 aa, synthetic construct
  REGION 1..11: note = FR4
RGPGTQVTVSS

SEQ ID NO: 93 - protein, 25 aa, synthetic construct
  REGION 1..25: note = FR1
EVQLVESGGEQVQPGSSLKLSCSVS

SEQ ID NO: 94 - protein, 8 aa, synthetic construct
  REGION 1..8: note = HCDR1
GLMISGHA

SEQ ID NO: 95 - protein, 25 aa, synthetic construct
  REGION 1..25: note = FR1
QVQLVESGGEQVQPGSSLKLSCSVS

SEQ ID NO: 96 - protein, 20 aa, synthetic construct
  REGION 1..20: note = HCDR3
ARVLSFKIYGGDKWALEWDY

SEQ ID NO: 97 - DNA, 951 bp, synthetic construct
  source 1..951: mol_type = other DNA
  misc_feature 1..951: note = huSOX2
atgtacaacatgatggagacggagctgaagccgccgggcccgcagcaaacttcggggggcggcggcggcaactccaccgcggcggcggccggcggcaaccagaaaaacagcccggaccgcgtcaagcggcccatgaatgccttcatggtgtggtcccgcgggcagcggcgcaagatggcccaggagaaccccaagatgcacaactcggagatcagcaagcgcctgggcgccgagtggaaacttttgtcggagacggagaagcggccgttcatcgacgaggctaagcggctgcgagcgctgcacatgaaggagcacccggattataaataccggccccggcggaaaaccaagacgctcatgaagaaggataagtacacgctgcccggcgggctgctggcccccggcggcaatagcatggcgagcggggtcggggtgggcgccggcctgggcgcgggcgtgaaccagcgcatggacagttacgcgcacatgaacggctggagcaacggcagctacagcatgatgcaggaccagctgggctacccgcagcacccgggcctcaatgcgcacggcgcagcgcagatgcagcccatgcaccgctacgacgtgagcgccctgcagtacaactccatgaccagctcgcagacctacatgaacggctcgcccacctacagcatgtcctactcgcagcagggcacccctggcatggctcttggctccatgggttcggtggtcaagtccgaggccagctccagcccccctgtggttacctcttcctcccactccagggcgccctgccaggccggggacctccgggacatgatcagcatgtatctccccggcgccgaggtgccggaacccgccgcccccagcagacttcacatgtcccagcactaccagagcggcccggtgcccggcacggccattaacggcacactgcccctctcacacatg

SEQ ID NO: 98 - DNA, 819 bp, synthetic construct
  source 1..819: mol_type = other DNA
  misc_feature 1..819: note = cynoSOX2
atgaatgccttcatggtgtggtcccgcgggcagcggcgcaaaatggcccaggagaaccccaagatgcacaactcggagatcagcaagcgcctcggagcagagtggaaacttttgtcggagacggagaagcggcccttcatcgacgaggctaagcggctgcgagcgctgcacatgaaggagcacccggattataaataccggccccggcggaaaaccaagacgctcatgaagaaggataagtacacgctgcccggcgggctgctggcccccggcggcaacagcatggcgagcggggtcggggtgggcgccggcctgggcgcgggcgtgaaccagcgcatggacagttacgcgcatatgaacggctggagcaacggcagctacagcatgatgcaggaccagctgggctaccctcagcacccgggcctcaacgcgcacggcgcagcgcagatgcagcccatgcaccgctacgacgtgagcgcactgcagtacaactccatgaccagctcgcagacctacatgaacggctcgcccacctacagcatgtcctactcgcagcagggcacccctggcatggctcttggttccatgggttcggtggtcaagtccgaggccagctccagcccccctgtggttacctcttcctcccactccagggcgccctgccaggccggggacctccgggacatgatcagcatgtatctccccggcgccgaggtgccggaacccgccgcccccagcagactgcacatgtcccagcactaccagagcggcccggtgcccggcacggccattaacggcacactgcccctctcgcacatg

SEQ ID NO: 99 - DNA, 1338 bp, synthetic construct
  source 1..1338: mol_type = other DNA
  misc_feature 1..1338: note = huSOX3
atgcgacctgttcgagagaactcatcaggtgcgagaagcccgcgggttcctgctgatttggcgcggagcattttgataagcctacccttcccgccggactcgctggcccacaggcccccaagctccgctccgacggagtcccagggccttttcaccgtggccgctccagccccgggagcgccttctcctcccgccacgctggcgcaccttcttcccgccccggcaatgtacagccttctggagactgaactcaagaaccccgtagggacacccacacaagcggcgggcaccggcggccccgcagccccgggaggcgcaggcaagagtagtgcgaacgcagccggcggcgcgaactcgggcggcggcagcagcggtggtgcgagcggaggtggcgggggtacagaccaggaccgtgtgaaacggcccatgaacgccttcatggtatggtcccgcgggcagcggcgcaaaatggccctggagaaccccaagatgcacaattctgagatcagcaagcgcttgggcgccgactggaaactgctgaccgacgccgagaagcgaccattcatcgacgaggccaagcgacttcgcgccgtgcacatgaaggagtatccggactacaagtaccgaccgcgccgcaagaccaagacgctgctcaagaaagataagtactccctgcccagcggcctcctgcctcccggtgccgcggccgccgccgccgctgccgcggccgcagccgctgccgccagcagtccggtgggcgtgggccagcgcctggacacgtacacgcacgtgaacggctgggccaacggcgcgtactcgctggtgcaggagcagctgggctacgcgcagcccccgagcatgagcagcccgccgccgccgcccgcgctgccgccgatgcaccgctacgacatggccggcctgcagtacagcccaatgatgccgcccggcgctcagagctacatgaacgtcgctgccgcggccgccgccgcctcgggctacgggggcatggcgccctcagccacagcagccgcggccgccgcctacgggcagcagcccgccaccgccgcggccgcagctgcggccgcagccgccatgagcctgggccccatgggctcggtagtgaagtctgagcccagctcgccgccgcccgccatcgcatcgcactctcagcgcgcgtgcctcggcgacctgcgcgacatgatcagcatgtacctgccacccggcggggacgcggccgacgccgcctctccgctgcccggcggtcgcctgcacggcgtgcaccagcactaccagggcgccgggactgcagtcaacggaacggtgccgctgacccacatc

SEQ ID NO: 100 - DNA, 558 bp, synthetic construct
  source 1..558: mol_type = other DNA
  misc_feature 1..558: note = Human SOX2 135-317
atgggtggcaatagcatggcgtctggtgttggtgtaggtgctggcctgggtgcaggtgtgaaccaacgtatggacagctatgctcacatgaatggctggagcaacggttcttacagcatgatgcaagatcagcttggctatccgcagcaccctggtctgaatgcacatggtgcagctcagatgcaacctatgcatcgttacgatgtatctgctctgcagtacaacagcatgactagctctcagacctatatgaatggctctccaacctacagcatgtcttactctcagcaaggtacccctggcatggctcttggtagcatgggtagcgttgtcaagtctgaagcaagctctagcccacctgtagttacttctagctctcactctcgtgctccatgtcaagcaggtgatttacgcgatatgatcagcatgtatcttccaggtgctgaagtacctgaacctgcagcacctagccgtctgcacatgtctcaacactatcagagcggccctgttccaggtactgctatcaatggtaccttgccactgtctcacatgactcgt

SEQ ID NO: 101 - DNA, 354 bp, synthetic construct
  source 1..354: mol_type = other DNA
  misc_feature 1..354: note = S14
caggtgaagctggaggagagcggcggcggcagcgtgcagaccggcggcagcctgaggctgacctgcgccgccagcggcagcatcttcagcatgaacaggatgggctggttcaggcaggcccccggcaaggagagggagctggtggccgtgatcgacagcaagaggaacaagacccactacgccgacagcgtgaagggcaggttcaccatcagcagggacaacgccaagaacaccgtggacctccagatgaacagcctgaagcccgaggacaccgccatctactactgcaccgcctggaccggcaggccccccaggggctactggggccagggcacccaggtgaccgtgagcagc

SEQ ID NO: 102 - DNA, 345 bp, synthetic construct
  source 1..345: mol_type = other DNA
  misc_feature 1..345: note = 1A5
gaagtgcagctggtggaaagcggcggcggcctggtgcagccgggcggcagcctgcgcctgagctgcgcggcgagcggcagcacctataccacctatagcatgggctggtttcgccaggcgccgggcaaagaacgcgaatttgtgggcgcgattcattggagcggcggccgcacctattatgcggatagcgtgaaaggccgctttaccattagcgcggataacagcaaaaacaccgcgtatctgcagatgaacagcctgaaaccggaagataccgcggtgtattattgcgcgagccgcgtggatgatcgcgtgtggggccagggcaccctggtgaccgtgagcagc

SEQ ID NO: 103 - DNA, 345 bp, synthetic construct
  source 1..345: mol_type = other DNA
  misc_feature 1..345: note = 1A9
gaagtgcagctggtggaaagcggcggcggcctggtgcagccgggcggcagcctgcgcctgagctgcgcggcgagcggccgcacctttagcacctatagcatgggctggtttcgccaggcgccgggcaaagaacgcgaatttgtggcggcgattcgctggaccgcgggcaccacctattatgcggatagcgtgaaaggccgctttaccattagcgcggataacagcaaaaacaccgcgtatctgcagatgaacagcctgaaaccggaagataccgcggtgtattattgcgcgagccgcgtggatgatcgcgtgtggggccagggcaccctggtgaccgtgagcagc

SEQ ID NO: 104 - DNA, 345 bp, synthetic construct
  source 1..345: mol_type = other DNA
  misc_feature 1..345: map = 1A11
gaagtgcagctggtggaaagcggcggcggcctggtgcagccgggcggcagcctgcgcctgagctgcgcggcgagcggcagcacctataccacctatagcatgggctggtttcgccaggcgccgggcaaagaacgcgaatttgtggcggcgattcactggagcggcggcggcacctattatgcggatagcgtgaaaggccgctttaccattagcgcggataacagcaaaaacaccgcgtatctgcagatgaacagcctgaaaccggaagataccgcggtgtattattgcgcgagccgcgtggatgatcgcgtgtggggccagggcaccctggtgaccgtgagcagc

SEQ ID NO: 105 - DNA, 348 bp, synthetic construct
  source 1..348: mol_type = other DNA
  misc_feature 1..348: note = 1B9
gaagtgcagctggtggaaagcggcggcggcctggtgcagccgggcggcagcctgcgcctgagctgcgcggcgagcggcctgacctttagcacctatagcatgggctggtttcgccaggcgccgggcaaagaacgcgaatttgtggcggcgattacctggaacagcggccgccgcacctattatgcggatagcgtgaaaggccgctttaccattagcgcggataacagcaaaaacaccgcgtatctgcagatgaacagcctgaaaccggaagataccgcggtgtattattgcgcgagccgcgtggatgatcgcgtgtggggccagggcaccctggtgaccgtgagcagc

SEQ ID NO: 106 - DNA, 345 bp, synthetic construct
  source 1..345: mol_type = other DNA
  misc_feature 1..345: note = 1C2
gaagtgcagctggtggaaagcggcggcggcctggtgcagccgggcggcagcctgcgcctgagctgcgcggcgagcggcagcacctataccacctatagcatgggctggtttcgccaggcgccgggcaaagaacgcgaatttgtggcggcgattcgctggagcggcggcaccacctattatgcggatagcgtgaaaggccgctttaccattagcgcggataacagcaaaaacaccgcgtatctgcagatgaacagcctgaaaccggaagataccgcggtgtattattgcgcgagccgcgtggatgatcgcgtgtggggccagggcaccctggtgaccgtgagcagc

SEQ ID NO: 107 - DNA, 345 bp, synthetic construct
  source 1..345: mol_type = other DNA
  misc_feature 1..345: note = 1C11
gaagtgcagctggtggaaagcggcggcggcctggtgcagccgggcggcagcctgcgcctgagctgcgcggcgagcggcagcacctataccacctatagcatgggctggtttcgccaggcgccgggcaaagaacgcgaatttgtgggggcgattcgctggagcggcggcaccacctattatgcggatagcgtgaaaggccgctttaccattagcgcggataacagcaaaaacaccgcgtatctgcagatgaacagcctgaaaccggaagataccgcggtgtattattgcgcgagccgcgtggatgatcgcgtgtggggccagggcaccctggtgaccgtgagcagc

SEQ ID NO: 108 - DNA, 345 bp, synthetic construct
  source 1..345: mol_type = other DNA
  misc_feature 1..345: note = 1C12
gaagtgcagctggtggaaagcggcggcggcctggtgcagccgggcggcagcctgcgcctgagctgcgcggcgagcggcagcacctataccacctatagcatgggctggtttcgccaggcgccgggcaaagaacgcgaatttgtggcggcgattcgctggagcggcggcagcacccattatgcggatagcgtgaaaggccgctttaccattagcgcggataacagcaaaaacaccgcgtatctgcagatgaacagcctgaaaccggaagataccgcggtgtattattgcgcgagccgcgtggatgatcgcgtgtggggccagggcaccctggtgaccgtgagcagc

SEQ ID NO: 109 - DNA, 357 bp, synthetic construct
  source 1..357: mol_type = other DNA
  misc_feature 1..357: note = 1C4
gaagtgcagctggtggaaagcggcggcggcctggtgcagccgggcggcagcctgcgcctgagctgcgcggcgagcggcggcggctttcgcggcaacgcggtgatgggctggtttcgccaggcgccgggcaaagaacgcgaactggtggcggcgattcgcggcagcggcgaagatacctattatgcggatagcgtgaaaggccgctttaccattagcgcggataacagcaaaaacaccgcgtatctgcagatgaacagcctgaaaccggaagataccgcggtgtattattgtgctggtgggtggcggcgtgggtatttccaggattggggccagggcaccctggtgaccgtgagcagc

SEQ ID NO: 110 - DNA, 354 bp, synthetic construct
  source 1..354: mol_type = other DNA
  misc_feature 1..354: note = 2E8
gaagtgcagctggtggaaagcggcggcggcctggtgcagccgggcggcagcctgcgcctgagctgcgcggcgagcggctttaccctggattattatggcatgggctggtttcgccaggcgccgggcaaagaacgcgaatttgtggcggcgattagccgcagcggcggcagcaccgtgtatgcggatagcgtgaaaggccgctttaccattagcgcggataacagcaaaaacaccgcgtatctgcagatgaacagcctgaaaccggaagataccgcggtgtattattgtgcacgcgaagttgtacgtggtggtattaattattggggccagggcaccctggtgaccgtgagcagc

SEQ ID NO: 111 - DNA, 378 bp, synthetic construct
  source 1..378: mol_type = other DNA
  misc_feature 1..378: note = 3F11
gatgtgcagctggtggagtctgggggaggcttggtgcagcctggggggtctctgagactctcctgtgcgacctccggattcaccttcagtagctcgaccatgagctgggtccgccaggttcctggcgcggggcctgaatgggttgcggttgataatcctggcggcaagaagaactacattgattccgtcgcgggccgattcaccatcgccagagacaacgacgcgaattccctgtctctggtgatgaatggcctgagacccgaggacacggcccgatatttctgcgcgcgagtattgtcctttaagatctacgagggcgataagtgggccctggagtgggactaccggggtccggggacccaggtcaccgtctcgtcg

SEQ ID NO: 112 - DNA, 378 bp, synthetic construct
  source 1..378: mol_type = other DNA
  misc_feature 1..378: note = 3A2
gaggtgcagttggtggagtctgggggagaacaggtgcagcctgggagctccctgaaactctcctgttcagtctctggattgatgatcagcggtcacgccatgagctgggtccgccaggttcctggcgcggggcccgaatgggttgcggttgataatcctggcggcaagaagaactacattgattccgtcgcgggccgattcaccatcgccagagacaacgacgcgaactccctgtctctggtgatgaatggcctgagacccgaggacacggcccgatatttctgcgcgcgagtattgtcctttaagatctacgagggcgataagtgggccctggagtgggactaccggggtccggggacccaggtcaccgtctcctca

SEQ ID NO: 113 - DNA, 378 bp, synthetic construct
  source 1..378: mol_type = other DNA
  misc_feature 1..378: note = 3H9
caagtgcagctggtggagtctgggggagaacaggtgcagcctgggagctccctgaaactctcctgttcagtctctggattgatgatcagcggtcacgccatgagctgggtccgccaggttcctggcgcggggcctgaatgggttgcggttgataatcctggcggcaagaagaactacattgattccgtcgcgggccgattcaccatcgccagagacaacgacgcgaattccctgtctctggtgatgaatggcctgagacccgaggacacggcccgatatttctgcgcgcgagtattgtcctttaagatctacgggggcgataagtgggccctggagtgggactaccggggtccggggacccaggtcaccgtctcgtcg

SEQ ID NO: 114 - DNA, 786 bp, synthetic construct
  source 1..786: mol_type = other DNA
  misc_feature 1..786: note = bTrCP190-228
gacccggccgaggcggtgctgcaagagaaggcactcaagtttatgaactcctcagagagagaagactgtaataatggcgaaccccctaggaagataataccagagaagaactcacttagacagacatacaacagctgtgccagactctgcttaaaccaagaaacagtatgtttagcaagcactgctatgaagactgagaattgtgtggccaaaacaaaacttgccaatggcacttccagtatgattgtgcccaagcaacggaaactctcagcaagctatgaaaaggaaaaggaactgtgtgtcaaatactttgagcagtggtcagagtcagatcaagtggaatttgtggaacatcttatatcccaaatgtgtcattaccaacatgggcacataaactcgtatcttaaacctatgttgcagagagatttcataactgctctgccagctcggggattggatcatattgctgagaacattctgtcatacctggatgccaaatcactatgtgctgctgaacttgtgtgcaaggaatggtaccgagtgacctctgatggcatgctgtggaagaagcttatcgagagaatggtcaggacagattctctgtggagaggcctggcagaacgaagaggatggggacagtatttattcaaaaacaaacctcctgacgggaatgctcctcccaactctttttatagagcactttatcctaaaattatacaagacattgagacaatagaatctaattggagatgtggaagacatagtttacagaggattcactgccga

SEQ ID NO: 115 - DNA, 525 bp, synthetic construct
  source 1..525: mol_type = other DNA
  misc_feature 1..525: note = SKP2 2-176
cacaggaagcacctccaggagattccagacctgagtagcaacgttgccaccagcttcacgtggggatgggattccagcaagacttctgaactgctgtcaggcatgggggtctccgccctggagaaagaggagcccgacagtgagaacatcccccaggaactgctctcaaacctgggccacccggagagccccccacggaaacggctgaagagcaaagggagtgacaaagactttgtgattgtccgcaggcctaagctaaatcgagagaactttccaggtgtttcatgggactcccttccggatgagctgctcttgggaatcttttcctgtctgtgcctccctgagctgctaaaggtctctggtgtttgtaagaggtggtatcgcctagcgtctgatgagtctctatggcagaccttagacctcacaggtaaaaatctgcacccggatgtgactggtcggttgctgtctcaaggggtgattgccttccgctgcccacgatcatttatggaccaaccattggctgaa

SEQ ID NO: 116 - DNA, 186 bp, synthetic construct
  source 1..186: mol_type = other DNA
  misc_feature 1..186: note = VHL152-213
acactgccagtgtatactctgaaagagcgatgcctccaggttgtccggagcctagtcaagcctgagaattacaggagactggacatcgtcaggtcgctctacgaagatctggaagaccacccaaatgtgcagaaagacctggagcggctgacacaggagcgcattgcacatcaacggatgggagat

SEQ ID NO: 117 - DNA, 624 bp, synthetic construct
  source 1..624: mol_type = other DNA
  misc_feature 1..624: note = SPOP167-374
tctgtcaacatttctggccagaataccatgaacatggtaaaggttcctgagtgccggctggcagatgagttaggaggactgtgggagaactcccggttcacagactgctgcttgtgtgttgccggccaggagttccaggctcacaaggctatcttagcagctcgttctccggtttttagtgccatgtttgaacatgaaatggaggagagcaaaaagaatcgagttgaaatcaatgatgtggagcctgaagtttttaaggaaatgatgtgcttcatttacacggggaaggctccaaacctcgacaaaatggctgatgatttgctggcagctgctgacaagtatgccctggagcgcttaaaggtcatgtgtgaggatgccctctgtagtaacctgtccgtggagaacgcagctgaaattctcatcctggccgacctccacagtgcagatcagttgaaaactcaggcagtggatttcatcaactatcatgcttcggatgtcttggagacctctgggtggaagtcaatggtggtgtcacatccccacttggtggctgaggcataccgctctctggcttcagcacagtgcccttttctgggacccccacgcaaacgcctgaagcaatcc

SEQ ID NO: 118 - DNA, 168 bp, synthetic construct
  source 1..168: mol_type = other DNA
  misc_feature 1..168: note = SOCS2 143-198
ccccggaacggcactgttcacctttatctgaccaaaccgctctacacgtcagcaccatctctccagcatctctgtaggctcaccattaacaaatgtaccggtgccatctggggactgcctttaccaacaagactaaaagattacttggaagaatataaattccaggta

SEQ ID NO: 119 - DNA, 528 bp, synthetic construct
  source 1..528: mol_type = other DNA
  misc_feature 1..528: note = CHIP128-303
cggctgaacttcggggacgacatccccagcgctcttcgaatcgcgaagaagaagcgctggaacagcattgaggagcggcgcatccaccaggagagcgagctgcactcctacctctccaggctcattgccgcggagcgtgagagggagctggaagagtgccagcgaaaccacgagggtgatgaggacgacagccacgtccgggcccagcaggcctgcattgaggccaagcacgacaagtacatggcggacatggacgagcttttttctcaggtggatgagaagaggaagaagcgagacatccccgactacctgtgtggcaagatcagctttgagctgatgcgggagccgtgcatcacgcccagtggcatcacctacgaccgcaaggacatcgaggagcacctccagcgtgtgggtcattttgaccccgtgacccggagccccctgacccaggaacagctcatccccaacttggctatgaaggaggttattgacgcattcatctctgagaatggctgggtggaggactac

SEQ ID NO: 120 - DNA, 339 bp, synthetic construct
  source 1..339: mol_type = other DNA
  misc_feature 1..339: note = DDB2 2-114
gctcccaagaaacgcccagaaacccagaagacctccgagattgtattacgccccaggaacaagaggagcaggagtcccctggagctggagcccgaggccaagaagctctgtgcgaagggctccggtcctagcagaagatgtgactcagactgcctctgggtggggctggctggcccacagatcctgccaccatgccgcagcatcgtcaggaccctccaccagcataagctgggcagagcttcctggccatctgtccagcaggggctccagcagtcctttttgcacactctggattcttaccggatattacaaaaggctgccccctttgacaggagggct

SEQ ID NO: 121 - DNA, 957 bp, synthetic construct
  source 1..957: mol_type = other DNA
  misc_feature 1..957: note = CRBN2-320
gccggcgaaggagatcagcaggacgctgcgcacaacatgggcaaccacctgccgctcctgccagcagagagtgaggaagaagatgaaatggaagttgaagaccaggatagtaaagaagccaaaaaaccaaacatcataaattttgacaccagtctgccgacatcacatacatacctaggtgctgatatggaagaatttcatggcaggactttgcacgatgacgacagctgtcaggtgattccagttcttccacaagtgatgatgatcctgattcccggacagacattacctcttcagctttttcaccctcaagaagtcagtatggtgcggaatttaattcagaaagatagaacctttgctgttcttgcatacagcaatgtacaggaaagggaagcacagtttggaacaacagcagagatatatgcctatcgagaagaacaggattttggaattgagatagtgaaagtgaaagcaattggaagacaaaggttcaaagtccttgagctaagaacacagtcagatggaatccagcaagctaaagtgcaaattcttcccgaatgtgtgttgccttcaaccatgtcagcagttcaattagaatccctcaataagtgccagatatttccttcaaaacctgtctcaagagaagaccaatgttcatataaatggtggcagaaataccagaagagaaagtttcattgtgcaaatctaacttcatggcctcgctggctgtattccttatatgatgctgagaccttaatggacagaatcaagaaacagctacgtgaatgggatgaaaatctaaaagatgattctcttccttcaaatccaatagatttttcttacagagtagctgcttgtcttcctattgatgatgtattgagaatacagctccttaaaattggcagtgctatccagcgacttcgctgtgaattagacattatgaataaatgtacttcc

SEQ ID NO: 122 - DNA, 210 bp, synthetic construct
  source 1..210: mol_type = other DNA
  misc_feature 1..210: note = ASB1 266-335
gtgaagtgggaatcgctgggcccagagtcgagaggaagaagaaaagtggaccctgaggccttgcaggtctttaaagaggccagaagtgttcccagaaccttgctgtgtctgtgccgtgtggctgtgagaagagctcttggcaaacaccggcttcatctgattccttcgctgcctctgccagaccccataaagaagtttctactccatgag

SEQ ID NO: 123 - DNA, 252 bp, synthetic construct
  source 1..252: mol_type = other DNA
  misc_feature 1..252: note = TRIM21 2-85
gcttcagcagcacgcttgacaatgatgtgggaggaggtcacatgccctatctgcctggaccccttcgtggagcctgtgagcatcgagtgtggccacagcttctgccaggaatgcatctctcaggttgggaaaggtgggggcagcgtctgtcctgtgtgccggcagcgctttctgctcaagaatctccggcccaatcgacagctagccaacatggtgaacaaccttaaagaaatcagccaggaggccagagag

SEQ ID NO: 124 - DNA, 360 bp, synthetic construct
  source 1..360: mol_type = other DNA
  misc_feature 1..360: note = RNF4 71-190
gacgaaagaagaagaccaaggaggaatgctaggaggctgccccaggaccatgctgacagctgtgtggtgagcagtgacgatgaggagttgtccagggacagagacgtatatgtgactacccatactcccagaaacgccagggatgagggcgctacaggcctcaggccctcaggtactgtcagttgtcccatctgcatggacggatactcagagatcgtgcagaatggacgtctcatcgtttccacagaatgcggccatgtcttctgtagccagtgcctccgtgattccctgaagaatgctaatacttgcccaacttgtaggaaaaagatcaaccacaaacggtaccaccccatttatata

SEQ ID NO: 125 - DNA, 438 bp, synthetic construct
  source 1..438: mol_type = other DNA
  misc_feature 1..438: note = UBE2D1 2-147
gccttgaagcgcatacaaaaagagctctctgaccttcaaagagacccaccagctcactgtagtgcaggtcccgtaggcgacgatctttttcactggcaggcgacgatcatgggcccaccagattccgcttaccagggcggggtttttttcctgaccgttcactttccaactgactatccatttaaacctccgaagatcgcattcacaaccaagatttatcatccgaatatcaatagtaatgggtctatctgtttggacatcctgcgaagccagtggtcccccgcgctgactgtcagtaaagttttgctctctatctgttcccttctgtgcgatccgaacccggacgaccctcttgtcccagacatcgcccagatatacaagtcagataaagaaaaatataatagacacgcccgcgaatggacgcagaagtatgcaatg

SEQ ID NO: 126 - DNA, 438 bp, synthetic construct
  source 1..438: mol_type = other DNA
  misc_feature 1..438: note = UBE2D4 2-147
gccctgaagcgcatccagaaggaattgactgatcttcagagggacccaccagcgcagtgctcagccggtccggtaggggacgaccttttccactggcaggccacaataatgggtccaaatgactctccataccaagggggtgtgtttttcctcaccatccatttcccgacagactatccattcaagccacctaaagtggctttcacgacaaaaatataccaccccaacattaacagcaacgggagcatttgtttggatatacttagatctcaatggagccccgcactgacggtgagtaaagtccttctgtccatttgtagccttttgtgtgacccgaaccctgatgacccacttgtaccagagattgcgcacacttacaaagcggatagagagaagtataaccgacttgcgagggagtggacgcaaaagtacgccatg

SEQ ID NO: 127 - DNA, 270 bp, synthetic construct
  source 1..270: mol_type = other DNA
  misc_feature 1..270: note = ZNFR1 138-227
agctcgcatagtggtttcaagtgccccatttgctccaagtctgtggcttctgacgagatggaaatgcactttataatgtgtttgagcaaacctcgcctctcctacaacgatgatgtgctgactaaagacgcgggtgagtgtgtgatctgcctggaggagctgctgcagggggacacgatagccaggctgccctgcctgtgcatctatcacaaaagctgcatagactcgtggtttgaagtgaacagatcttgtccggaacaccctgcggac

SEQ ID NO: 128 - DNA, 999 bp, synthetic construct
  source 1..999: mol_type = other DNA
  misc_feature 1..999: note = huSOX2.Myc
atgtacaacatgatggagacggagctgaagccgccgggcccgcagcaaacttcggggggcggcggcggcaactccaccgcggcggcggccggcggcaaccagaaaaacagcccggaccgcgtcaagcggcccatgaatgccttcatggtgtggtcccgcgggcagcggcgcaagatggcccaggagaaccccaagatgcacaactcggagatcagcaagcgcctgggcgccgagtggaaacttttgtcggagacggagaagcggccgttcatcgacgaggctaagcggctgcgagcgctgcacatgaaggagcacccggattataaataccggccccggcggaaaaccaagacgctcatgaagaaggataagtacacgctgcccggcgggctgctggcccccggcggcaatagcatggcgagcggggtcggggtgggcgccggcctgggcgcgggcgtgaaccagcgcatggacagttacgcgcacatgaacggctggagcaacggcagctacagcatgatgcaggaccagctgggctacccgcagcacccgggcctcaatgcgcacggcgcagcgcagatgcagcccatgcaccgctacgacgtgagcgccctgcagtacaactccatgaccagctcgcagacctacatgaacggctcgcccacctacagcatgtcctactcgcagcagggcacccctggcatggctcttggctccatgggttcggtggtcaagtccgaggccagctccagcccccctgtggttacctcttcctcccactccagggcgccctgccaggccggggacctccgggacatgatcagcatgtatctccccggcgccgaggtgccggaacccgccgcccccagcagacttcacatgtcccagcactaccagagcggcccggtgcccggcacggccattaacggcacactgcccctctcacacatgacgcgtacgcggccgctcgagcagaaactcatctcagaagaggatctg

SEQ ID NO: 129 - DNA, 1176 bp, synthetic construct
  source 1..1176: mol_type = other DNA
  misc_feature 1..1176: note = Flag tag-bTrCP190-228.GS.S14
gactacaaggacgacgatgacaagacgcgtgacccggccgaggcggtgctgcaagagaaggcactcaagtttatgaactcctcagagagagaagactgtaataatggcgaaccccctaggaagataataccagagaagaactcacttagacagacatacaacagctgtgccagactctgcttaaaccaagaaacagtatgtttagcaagcactgctatgaagactgagaattgtgtggccaaaacaaaacttgccaatggcacttccagtatgattgtgcccaagcaacggaaactctcagcaagctatgaaaaggaaaaggaactgtgtgtcaaatactttgagcagtggtcagagtcagatcaagtggaatttgtggaacatcttatatcccaaatgtgtcattaccaacatgggcacataaactcgtatcttaaacctatgttgcagagagatttcataactgctctgccagctcggggattggatcatattgctgagaacattctgtcatacctggatgccaaatcactatgtgctgctgaacttgtgtgcaaggaatggtaccgagtgacctctgatggcatgctgtggaagaagcttatcgagagaatggtcaggacagattctctgtggagaggcctggcagaacgaagaggatggggacagtatttattcaaaaacaaacctcctgacgggaatgctcctcccaactctttttatagagcactttatcctaaaattatacaagacattgagacaatagaatctaattggagatgtggaagacatagtttacagaggattcactgccgaggatcccaggtgaagctggaggagagcggcggcggcagcgtgcagaccggcggcagcctgaggctgacctgcgccgccagcggcagcatcttcagcatgaacaggatgggctggttcaggcaggcccccggcaaggagagggagctggtggccgtgatcgacagcaagaggaacaagacccactacgccgacagcgtgaagggcaggttcaccatcagcagggacaacgccaagaacaccgtggacctccagatgaacagcctgaagcccgaggacaccgccatctactactgcaccgcctggaccggcaggccccccaggggctactggggccagggcacccaggtgaccgtgagcagc

SEQ ID NO: 130 - DNA, 915 bp, synthetic construct
  source 1..915: mol_type = other DNA
  misc_feature 1..915: note = Flag tag-SKP22-176.GS.S14
gactacaaggacgacgatgacaagacgcgtcacaggaagcacctccaggagattccagacctgagtagcaacgttgccaccagcttcacgtggggatgggattccagcaagacttctgaactgctgtcaggcatgggggtctccgccctggagaaagaggagcccgacagtgagaacatcccccaggaactgctctcaaacctgggccacccggagagccccccacggaaacggctgaagagcaaagggagtgacaaagactttgtgattgtccgcaggcctaagctaaatcgagagaactttccaggtgtttcatgggactcccttccggatgagctgctcttgggaatcttttcctgtctgtgcctccctgagctgctaaaggtctctggtgtttgtaagaggtggtatcgcctagcgtctgatgagtctctatggcagaccttagacctcacaggtaaaaatctgcacccggatgtgactggtcggttgctgtctcaaggggtgattgccttccgctgcccacgatcatttatggaccaaccattggctgaaggatcccaggtgaagctggaggagagcggcggcggcagcgtgcagaccggcggcagcctgaggctgacctgcgccgccagcggcagcatcttcagcatgaacaggatgggctggttcaggcaggcccccggcaaggagagggagctggtggccgtgatcgacagcaagaggaacaagacccactacgccgacagcgtgaagggcaggttcaccatcagcagggacaacgccaagaacaccgtggacctccagatgaacagcctgaagcccgaggacaccgccatctactactgcaccgcctggaccggcaggccccccaggggctactggggccagggcacccaggtgaccgtgagcagc

SEQ ID NO: 131 - DNA, 576 bp, synthetic construct
  source 1..576: mol_type = other DNA
  misc_feature 1..576: note = Flag tag-S14.GS.VHL152-213
gactacaaggacgacgatgacaagacgcgtcaggtgaagctggaggagagcggcggcggcagcgtgcagaccggcggcagcctgaggctgacctgcgccgccagcggcagcatcttcagcatgaacaggatgggctggttcaggcaggcccccggcaaggagagggagctggtggccgtgatcgacagcaagaggaacaagacccactacgccgacagcgtgaagggcaggttcaccatcagcagggacaacgccaagaacaccgtggacctccagatgaacagcctgaagcccgaggacaccgccatctactactgcaccgcctggaccggcaggccccccaggggctactggggccagggcacccaggtgaccgtgagcagcggatccacactgccagtgtatactctgaaagagcgatgcctccaggttgtccggagcctagtcaagcctgagaattacaggagactggacatcgtcaggtcgctctacgaagatctggaagaccacccaaatgtgcagaaagacctggagcggctgacacaggagcgcattgcacatcaacggatgggagat

SEQ ID NO: 132 - DNA, 1014 bp, synthetic construct
  source 1..1014: mol_type = other DNA
  misc_feature 1..1014: note = Flag tag-S14.GS.SPOP167-374
gactacaaggacgacgatgacaagacgcgtcaggtgaagctggaggagagcggcggcggcagcgtgcagaccggcggcagcctgaggctgacctgcgccgccagcggcagcatcttcagcatgaacaggatgggctggttcaggcaggcccccggcaaggagagggagctggtggccgtgatcgacagcaagaggaacaagacccactacgccgacagcgtgaagggcaggttcaccatcagcagggacaacgccaagaacaccgtggacctccagatgaacagcctgaagcccgaggacaccgccatctactactgcaccgcctggaccggcaggccccccaggggctactggggccagggcacccaggtgaccgtgagcagcggatcctctgtcaacatttctggccagaataccatgaacatggtaaaggttcctgagtgccggctggcagatgagttaggaggactgtgggagaactcccggttcacagactgctgcttgtgtgttgccggccaggagttccaggctcacaaggctatcttagcagctcgttctccggtttttagtgccatgtttgaacatgaaatggaggagagcaaaaagaatcgagttgaaatcaatgatgtggagcctgaagtttttaaggaaatgatgtgcttcatttacacggggaaggctccaaacctcgacaaaatggctgatgatttgctggcagctgctgacaagtatgccctggagcgcttaaaggtcatgtgtgaggatgccctctgtagtaacctgtccgtggagaacgcagctgaaattctcatcctggccgacctccacagtgcagatcagttgaaaactcaggcagtggatttcatcaactatcatgcttcggatgtcttggagacctctgggtggaagtcaatggtggtgtcacatccccacttggtggctgaggcataccgctctctggcttcagcacagtgcccttttctgggacccccacgcaaacgcctgaagcaatcc

SEQ ID NO: 133 - DNA, 558 bp, synthetic construct
  source 1..558: mol_type = other DNA
  misc_feature 1..558: note = Flag tag-S14.GS.SOCS2 143-198
gactacaaggacgacgatgacaagacgcgtcaggtgaagctggaggagagcggcggcggcagcgtgcagaccggcggcagcctgaggctgacctgcgccgccagcggcagcatcttcagcatgaacaggatgggctggttcaggcaggcccccggcaaggagagggagctggtggccgtgatcgacagcaagaggaacaagacccactacgccgacagcgtgaagggcaggttcaccatcagcagggacaacgccaagaacaccgtggacctccagatgaacagcctgaagcccgaggacaccgccatctactactgcaccgcctggaccggcaggccccccaggggctactggggccagggcacccaggtgaccgtgagcagcggatccccccggaacggcactgttcacctttatctgaccaaaccgctctacacgtcagcaccatctctccagcatctctgtaggctcaccattaacaaatgtaccggtgccatctggggactgcctttaccaacaagactaaaagattacttggaagaatataaattccaggta

SEQ ID NO: 134 - DNA, 918 bp, synthetic construct
  source 1..918: mol_type = other DNA
  misc_feature 1..918: note = Flag tag-S14.GS.CHIP 128-303
gactacaaggacgacgatgacaagacgcgtcaggtgaagctggaggagagcggcggcggcagcgtgcagaccggcggcagcctgaggctgacctgcgccgccagcggcagcatcttcagcatgaacaggatgggctggttcaggcaggcccccggcaaggagagggagctggtggccgtgatcgacagcaagaggaacaagacccactacgccgacagcgtgaagggcaggttcaccatcagcagggacaacgccaagaacaccgtggacctccagatgaacagcctgaagcccgaggacaccgccatctactactgcaccgcctggaccggcaggccccccaggggctactggggccagggcacccaggtgaccgtgagcagcggatcccggctgaacttcggggacgacatccccagcgctcttcgaatcgcgaagaagaagcgctggaacagcattgaggagcggcgcatccaccaggagagcgagctgcactcctacctctccaggctcattgccgcggagcgtgagagggagctggaagagtgccagcgaaaccacgagggtgatgaggacgacagccacgtccgggcccagcaggcctgcattgaggccaagcacgacaagtacatggcggacatggacgagcttttttctcaggtggatgagaagaggaagaagcgagacatccccgactacctgtgtggcaagatcagctttgagctgatgcgggagccgtgcatcacgcccagtggcatcacctacgaccgcaaggacatcgaggagcacctccagcgtgtgggtcattttgaccccgtgacccggagccccctgacccaggaacagctcatccccaacttggctatgaaggaggttattgacgcattcatctctgagaatggctgggtggaggactac

SEQ ID NO: 135 - DNA, 729 bp, synthetic construct
  source 1..729: mol_type = other DNA
  misc_feature 1..729: note = Flag tag-DDB2 2-114.GS.S14
gactacaaggacgacgatgacaagacgcgtgctcccaagaaacgcccagaaacccagaagacctccgagattgtattacgccccaggaacaagaggagcaggagtcccctggagctggagcccgaggccaagaagctctgtgcgaagggctccggtcctagcagaagatgtgactcagactgcctctgggtggggctggctggcccacagatcctgccaccatgccgcagcatcgtcaggaccctccaccagcataagctgggcagagcttcctggccatctgtccagcaggggctccagcagtcctttttgcacactctggattcttaccggatattacaaaaggctgccccctttgacaggagggctggatcccaggtgaagctggaggagagcggcggcggcagcgtgcagaccggcggcagcctgaggctgacctgcgccgccagcggcagcatcttcagcatgaacaggatgggctggttcaggcaggcccccggcaaggagagggagctggtggccgtgatcgacagcaagaggaacaagacccactacgccgacagcgtgaagggcaggttcaccatcagcagggacaacgccaagaacaccgtggacctccagatgaacagcctgaagcccgaggacaccgccatctactactgcaccgcctggaccggcaggccccccaggggctactggggccagggcacccaggtgaccgtgagcagc

SEQ ID NO: 136 - DNA, 1347 bp, synthetic construct
  source 1..1347: mol_type = other DNA
  misc_feature 1..1347: note = Flag tag-CRBN2-320.GS.S14
gactacaaggacgacgatgacaagacgcgtgccggcgaaggagatcagcaggacgctgcgcacaacatgggcaaccacctgccgctcctgccagcagagagtgaggaagaagatgaaatggaagttgaagaccaggatagtaaagaagccaaaaaaccaaacatcataaattttgacaccagtctgccgacatcacatacatacctaggtgctgatatggaagaatttcatggcaggactttgcacgatgacgacagctgtcaggtgattccagttcttccacaagtgatgatgatcctgattcccggacagacattacctcttcagctttttcaccctcaagaagtcagtatggtgcggaatttaattcagaaagatagaacctttgctgttcttgcatacagcaatgtacaggaaagggaagcacagtttggaacaacagcagagatatatgcctatcgagaagaacaggattttggaattgagatagtgaaagtgaaagcaattggaagacaaaggttcaaagtccttgagctaagaacacagtcagatggaatccagcaagctaaagtgcaaattcttcccgaatgtgtgttgccttcaaccatgtcagcagttcaattagaatccctcaataagtgccagatatttccttcaaaacctgtctcaagagaagaccaatgttcatataaatggtggcagaaataccagaagagaaagtttcattgtgcaaatctaacttcatggcctcgctggctgtattccttatatgatgctgagaccttaatggacagaatcaagaaacagctacgtgaatgggatgaaaatctaaaagatgattctcttccttcaaatccaatagatttttcttacagagtagctgcttgtcttcctattgatgatgtattgagaatacagctccttaaaattggcagtgctatccagcgacttcgctgtgaattagacattatgaataaatgtacttccggatcccaggtgaagctggaggagagcggcggcggcagcgtgcagaccggcggcagcctgaggctgacctgcgccgccagcggcagcatcttcagcatgaacaggatgggctggttcaggcaggcccccggcaaggagagggagctggtggccgtgatcgacagcaagaggaacaagacccactacgccgacagcgtgaagggcaggttcaccatcagcagggacaacgccaagaacaccgtggacctccagatgaacagcctgaagcccgaggacaccgccatctactactgcaccgcctggaccggcaggccccccaggggctactggggccagggcacccaggtgaccgtgagcagc

SEQ ID NO: 137 - DNA, 600 bp, synthetic construct
  source 1..600: mol_type = other DNA
  misc_feature 1..600: note = Flag tag-S14.GS.ASB1 266-335
gactacaaggacgacgatgacaagacgcgtcaggtgaagctggaggagagcggcggcggcagcgtgcagaccggcggcagcctgaggctgacctgcgccgccagcggcagcatcttcagcatgaacaggatgggctggttcaggcaggcccccggcaaggagagggagctggtggccgtgatcgacagcaagaggaacaagacccactacgccgacagcgtgaagggcaggttcaccatcagcagggacaacgccaagaacaccgtggacctccagatgaacagcctgaagcccgaggacaccgccatctactactgcaccgcctggaccggcaggccccccaggggctactggggccagggcacccaggtgaccgtgagcagcggatccgtgaagtgggaatcgctgggcccagagtcgagaggaagaagaaaagtggaccctgaggccttgcaggtctttaaagaggccagaagtgttcccagaaccttgctgtgtctgtgccgtgtggctgtgagaagagctcttggcaaacaccggcttcatctgattccttcgctgcctctgccagaccccataaagaagtttctactccatgag

SEQ ID NO: 138 - DNA, 642 bp, synthetic construct
  source 1..642: mol_type = other DNA
  misc_feature 1..624: note = Flag tag-TRIM21 2-85.GS.S14
gactacaaggacgacgatgacaagacgcgtgcttcagcagcacgcttgacaatgatgtgggaggaggtcacatgccctatctgcctggaccccttcgtggagcctgtgagcatcgagtgtggccacagcttctgccaggaatgcatctctcaggttgggaaaggtgggggcagcgtctgtcctgtgtgccggcagcgctttctgctcaagaatctccggcccaatcgacagctagccaacatggtgaacaaccttaaagaaatcagccaggaggccagagagggatcccaggtgaagctggaggagagcggcggcggcagcgtgcagaccggcggcagcctgaggctgacctgcgccgccagcggcagcatcttcagcatgaacaggatgggctggttcaggcaggcccccggcaaggagagggagctggtggccgtgatcgacagcaagaggaacaagacccactacgccgacagcgtgaagggcaggttcaccatcagcagggacaacgccaagaacaccgtggacctccagatgaacagcctgaagcccgaggacaccgccatctactactgcaccgcctggaccggcaggccccccaggggctactggggccagggcacccaggtgaccgtgagcagc

SEQ ID NO: 139 - DNA, 750 bp, synthetic construct
  source 1..750: mol_type = other DNA
  misc_feature 1..750: note = Flag tag-S14.GS.RNF4 71-190
gactacaaggacgacgatgacaagacgcgtcaggtgaagctggaggagagcggcggcggcagcgtgcagaccggcggcagcctgaggctgacctgcgccgccagcggcagcatcttcagcatgaacaggatgggctggttcaggcaggcccccggcaaggagagggagctggtggccgtgatcgacagcaagaggaacaagacccactacgccgacagcgtgaagggcaggttcaccatcagcagggacaacgccaagaacaccgtggacctccagatgaacagcctgaagcccgaggacaccgccatctactactgcaccgcctggaccggcaggccccccaggggctactggggccagggcacccaggtgaccgtgagcagcggatccgacgaaagaagaagaccaaggaggaatgctaggaggctgccccaggaccatgctgacagctgtgtggtgagcagtgacgatgaggagttgtccagggacagagacgtatatgtgactacccatactcccagaaacgccagggatgagggcgctacaggcctcaggccctcaggtactgtcagttgtcccatctgcatggacggatactcagagatcgtgcagaatggacgtctcatcgtttccacagaatgcggccatgtcttctgtagccagtgcctccgtgattccctgaagaatgctaatacttgcccaacttgtaggaaaaagatcaaccacaaacggtaccaccccatttatata

SEQ ID NO: 140 - DNA, 600 bp, synthetic construct
  source 1..600: mol_type = other DNA
  misc_feature 1..600: note = Flag tag-3A2.GS.VHL152-213
gactacaaggacgacgatgacaagacgcgtgaggtgcaattggttgagtcaggaggtgagcaggtccaacctggtagttctttgaaattgagctgttcagtctcaggtctgatgatatcaggccacgcgatgagttgggtcaggcaagtaccgggggccgggcctgagtgggtcgcggtggataatccagggggtaaaaagaactatattgactcagttgctggcagatttacgattgctcgggacaacgatgcaaactctctgagcctcgttatgaacggtctgcggcctgaggacacagccaggtacttctgcgcccgagtattgagctttaagatatacgaaggagataaatgggctctggagtgggactatcgcgggccgggcacacaagtgacggtgtccagcggatccacactgccagtgtatactctgaaagagcgatgcctccaggttgtccggagcctagtcaagcctgagaattacaggagactggacatcgtcaggtcgctctacgaagatctggaagaccacccaaatgtgcagaaagacctggagcggctgacacaggagcgcattgcacatcaacggatgggagat

SEQ ID NO: 141 - DNA, 1038 bp, synthetic construct
  source 1..1038: mol_type = other DNA
  misc_feature 1..1038: note = Flag tag-3A2.GS.SPOP167-374
gactacaaggacgacgatgacaagacgcgtgaggtgcaattggttgagtcaggaggtgagcaggtccaacctggtagttctttgaaattgagctgttcagtctcaggtctgatgatatcaggccacgcgatgagttgggtcaggcaagtaccgggggccgggcctgagtgggtcgcggtggataatccagggggtaaaaagaactatattgactcagttgctggcagatttacgattgctcgggacaacgatgcaaactctctgagcctcgttatgaacggtctgcggcctgaggacacagccaggtacttctgcgcccgagtattgagctttaagatatacgaaggagataaatgggctctggagtgggactatcgcgggccgggcacacaagtgacggtgtccagcggatcctctgtcaacatttctggccagaataccatgaacatggtaaaggttcctgagtgccggctggcagatgagttaggaggactgtgggagaactcccggttcacagactgctgcttgtgtgttgccggccaggagttccaggctcacaaggctatcttagcagctcgttctccggtttttagtgccatgtttgaacatgaaatggaggagagcaaaaagaatcgagttgaaatcaatgatgtggagcctgaagtttttaaggaaatgatgtgcttcatttacacggggaaggctccaaacctcgacaaaatggctgatgatttgctggcagctgctgacaagtatgccctggagcgcttaaaggtcatgtgtgaggatgccctctgtagtaacctgtccgtggagaacgcagctgaaattctcatcctggccgacctccacagtgcagatcagttgaaaactcaggcagtggatttcatcaactatcatgcttcggatgtcttggagacctctgggtggaagtcaatggtggtgtcacatccccacttggtggctgaggcataccgctctctggcttcagcacagtgcccttttctgggacccccacgcaaacgcctgaagcaatcc

SEQ ID NO: 142 - DNA, 582 bp, synthetic construct
  source 1..582: mol_type = other DNA
  misc_feature 1..582: note = Flag tag-3A2.GS.SOCS2 143-198
gactacaaggacgacgatgacaagacgcgtgaggtgcaattggttgagtcaggaggtgagcaggtccaacctggtagttctttgaaattgagctgttcagtctcaggtctgatgatatcaggccacgcgatgagttgggtcaggcaagtaccgggggccgggcctgagtgggtcgcggtggataatccagggggtaaaaagaactatattgactcagttgctggcagatttacgattgctcgggacaacgatgcaaactctctgagcctcgttatgaacggtctgcggcctgaggacacagccaggtacttctgcgcccgagtattgagctttaagatatacgaaggagataaatgggctctggagtgggactatcgcgggccgggcacacaagtgacggtgtccagcggatccccccggaacggcactgttcacctttatctgaccaaaccgctctacacgtcagcaccatctctccagcatctctgtaggctcaccattaacaaatgtaccggtgccatctggggactgcctttaccaacaagactaaaagattacttggaagaatataaattccaggta

SEQ ID NO: 143 - DNA, 942 bp, synthetic construct
  source 1..942: mol_type = other DNA
  misc_feature 1..942: note = Flag tag-3A2.GS.CHIP128-303
gactacaaggacgacgatgacaagacgcgtgaggtgcaattggttgagtcaggaggtgagcaggtccaacctggtagttctttgaaattgagctgttcagtctcaggtctgatgatatcaggccacgcgatgagttgggtcaggcaagtaccgggggccgggcctgagtgggtcgcggtggataatccagggggtaaaaagaactatattgactcagttgctggcagatttacgattgctcgggacaacgatgcaaactctctgagcctcgttatgaacggtctgcggcctgaggacacagccaggtacttctgcgcccgagtattgagctttaagatatacgaaggagataaatgggctctggagtgggactatcgcgggccgggcacacaagtgacggtgtccagcggatcccggctgaacttcggggacgacatccccagcgctcttcgaatcgcgaagaagaagcgctggaacagcattgaggagcggcgcatccaccaggagagcgagctgcactcctacctctccaggctcattgccgcggagcgtgagagggagctggaagagtgccagcgaaaccacgagggtgatgaggacgacagccacgtccgggcccagcaggcctgcattgaggccaagcacgacaagtacatggcggacatggacgagcttttttctcaggtggatgagaagaggaagaagcgagacatccccgactacctgtgtggcaagatcagctttgagctgatgcgggagccgtgcatcacgcccagtggcatcacctacgaccgcaaggacatcgaggagcacctccagcgtgtgggtcattttgaccccgtgacccggagccccctgacccaggaacagctcatccccaacttggctatgaaggaggttattgacgcattcatctctgagaatggctgggtggaggactac

SEQ ID NO: 144 - DNA, 624 bp, synthetic construct
  source 1..624: mol_type = other DNA
  misc_feature 1..624: note = Flag tag-3A2GS.ASB1 266-335
gactacaaggacgacgatgacaagacgcgtgaggtgcaattggttgagtcaggaggtgagcaggtccaacctggtagttctttgaaattgagctgttcagtctcaggtctgatgatatcaggccacgcgatgagttgggtcaggcaagtaccgggggccgggcctgagtgggtcgcggtggataatccagggggtaaaaagaactatattgactcagttgctggcagatttacgattgctcgggacaacgatgcaaactctctgagcctcgttatgaacggtctgcggcctgaggacacagccaggtacttctgcgcccgagtattgagctttaagatatacgaaggagataaatgggctctggagtgggactatcgcgggccgggcacacaagtgacggtgtccagcggatccgtgaagtgggaatcgctgggcccagagtcgagaggaagaagaaaagtggaccctgaggccttgcaggtctttaaagaggccagaagtgttcccagaaccttgctgtgtctgtgccgtgtggctgtgagaagagctcttggcaaacaccggcttcatctgattccttcgctgcctctgccagaccccataaagaagtttctactccatgag

SEQ ID NO: 145 - DNA, 666 bp, synthetic construct
  source 1..666: mol_type = other DNA
  misc_feature 1..666: note = Flag tag-TRIM21 2-85.GS.3A2
gactacaaggacgacgatgacaagacgcgtgcttcagcagcacgcttgacaatgatgtgggaggaggtcacatgccctatctgcctggaccccttcgtggagcctgtgagcatcgagtgtggccacagcttctgccaggaatgcatctctcaggttgggaaaggtgggggcagcgtctgtcctgtgtgccggcagcgctttctgctcaagaatctccggcccaatcgacagctagccaacatggtgaacaaccttaaagaaatcagccaggaggccagagagggatccgaggtgcaattggttgagtcaggaggtgagcaggtccaacctggtagttctttgaaattgagctgttcagtctcaggtctgatgatatcaggccacgcgatgagttgggtcaggcaagtaccgggggccgggcctgagtgggtcgcggtggataatccagggggtaaaaagaactatattgactcagttgctggcagatttacgattgctcgggacaacgatgcaaactctctgagcctcgttatgaacggtctgcggcctgaggacacagccaggtacttctgcgcccgagtattgagctttaagatatacgaaggagataaatgggctctggagtgggactatcgcgggccgggcacacaagtgacggtgtccagc

SEQ ID NO: 146 - DNA, 774 bp, synthetic construct
  source 1..774: mol_type = other DNA
  misc_feature 1..774: note = Flag tag-3A2.GS.RNF4 71-190
gactacaaggacgacgatgacaagacgcgtgaggtgcaattggttgagtcaggaggtgagcaggtccaacctggtagttctttgaaattgagctgttcagtctcaggtctgatgatatcaggccacgcgatgagttgggtcaggcaagtaccgggggccgggcctgagtgggtcgcggtggataatccagggggtaaaaagaactatattgactcagttgctggcagatttacgattgctcgggacaacgatgcaaactctctgagcctcgttatgaacggtctgcggcctgaggacacagccaggtacttctgcgcccgagtattgagctttaagatatacgaaggagataaatgggctctggagtgggactatcgcgggccgggcacacaagtgacggtgtccagcggatccgacgaaagaagaagaccaaggaggaatgctaggaggctgccccaggaccatgctgacagctgtgtggtgagcagtgacgatgaggagttgtccagggacagagacgtatatgtgactacccatactcccagaaacgccagggatgagggcgctacaggcctcaggccctcaggtactgtcagttgtcccatctgcatggacggatactcagagatcgtgcagaatggacgtctcatcgtttccacagaatgcggccatgtcttctgtagccagtgcctccgtgattccctgaagaatgctaatacttgcccaacttgtaggaaaaagatcaaccacaaacggtaccaccccatttatata

SEQ ID NO: 147 - DNA, 852 bp, synthetic construct
  source 1..852: mol_type = other DNA
  misc_feature 1..852: note = Flag tag-3A2.GS.UBE2D1 2-147
gactacaaggacgacgatgacaagacgcgtgaggtgcaattggttgagtcaggaggtgagcaggtccaacctggtagttctttgaaattgagctgttcagtctcaggtctgatgatatcaggccacgcgatgagttgggtcaggcaagtaccgggggccgggcctgagtgggtcgcggtggataatccagggggtaaaaagaactatattgactcagttgctggcagatttacgattgctcgggacaacgatgcaaactctctgagcctcgttatgaacggtctgcggcctgaggacacagccaggtacttctgcgcccgagtattgagctttaagatatacgaaggagataaatgggctctggagtgggactatcgcgggccgggcacacaagtgacggtgtccagcggatccgccttgaagcgcatacaaaaagagctctctgaccttcaaagagacccaccagctcactgtagtgcaggtcccgtaggcgacgatctttttcactggcaggcgacgatcatgggcccaccagattccgcttaccagggcggggtttttttcctgaccgttcactttccaactgactatccatttaaacctccgaagatcgcattcacaaccaagatttatcatccgaatatcaatagtaatgggtctatctgtttggacatcctgcgaagccagtggtcccccgcgctgactgtcagtaaagttttgctctctatctgttcccttctgtgcgatccgaacccggacgaccctcttgtcccagacatcgcccagatatacaagtcagataaagaaaaatataatagacacgcccgcgaatggacgcagaagtatgcaatg

SEQ ID NO: 148 - DNA, 852 bp, synthetic construct
  source 1..852: mol_type = other DNA
  misc_feature 1..852: note = Flag tag-3A2.GS.UBE2D4 2-147
gactacaaggacgacgatgacaagacgcgtgaggtgcaattggttgagtcaggaggtgagcaggtccaacctggtagttctttgaaattgagctgttcagtctcaggtctgatgatatcaggccacgcgatgagttgggtcaggcaagtaccgggggccgggcctgagtgggtcgcggtggataatccagggggtaaaaagaactatattgactcagttgctggcagatttacgattgctcgggacaacgatgcaaactctctgagcctcgttatgaacggtctgcggcctgaggacacagccaggtacttctgcgcccgagtattgagctttaagatatacgaaggagataaatgggctctggagtgggactatcgcgggccgggcacacaagtgacggtgtccagcggatccgccctgaagcgcatccagaaggaattgactgatcttcagagggacccaccagcgcagtgctcagccggtccggtaggggacgaccttttccactggcaggccacaataatgggtccaaatgactctccataccaagggggtgtgtttttcctcaccatccatttcccgacagactatccattcaagccacctaaagtggctttcacgacaaaaatataccaccccaacattaacagcaacgggagcatttgtttggatatacttagatctcaatggagccccgcactgacggtgagtaaagtccttctgtccatttgtagccttttgtgtgacccgaaccctgatgacccacttgtaccagagattgcgcacacttacaaagcggatagagagaagtataaccgacttgcgagggagtggacgcaaaagtacgccatg

SEQ ID NO: 149 - DNA, 684 bp, synthetic construct
  source 1..684: mol_type = other DNA
  misc_feature 1..684: note = Flag tag-3A2.GS.ZNFR1 138-227
gactacaaggacgacgatgacaagacgcgtgaggtgcaattggttgagtcaggaggtgagcaggtccaacctggtagttctttgaaattgagctgttcagtctcaggtctgatgatatcaggccacgcgatgagttgggtcaggcaagtaccgggggccgggcctgagtgggtcgcggtggataatccagggggtaaaaagaactatattgactcagttgctggcagatttacgattgctcgggacaacgatgcaaactctctgagcctcgttatgaacggtctgcggcctgaggacacagccaggtacttctgcgcccgagtattgagctttaagatatacgaaggagataaatgggctctggagtgggactatcgcgggccgggcacacaagtgacggtgtccagcggatccagctcgcatagtggtttcaagtgccccatttgctccaagtctgtggcttctgacgagatggaaatgcactttataatgtgtttgagcaaacctcgcctctcctacaacgatgatgtgctgactaaagacgcgggtgagtgtgtgatctgcctggaggagctgctgcagggggacacgatagccaggctgccctgcctgtgcatctatcacaaaagctgcatagactcgtggtttgaagtgaacagatcttgtccggaacaccctgcggac

SEQ ID NO: 150 - DNA, 1011 bp, synthetic construct
  source 1..1011: mol_type = other DNA
  misc_feature 1..1011: note = huSOX2.V5
atgtacaacatgatggagacggagctgaagccgccgggcccgcagcaaacttcggggggcggcggcggcaactccaccgcggcggcggccggcggcaaccagaaaaacagcccggaccgcgtcaagcggcccatgaatgccttcatggtgtggtcccgcgggcagcggcgcaagatggcccaggagaaccccaagatgcacaactcggagatcagcaagcgcctgggcgccgagtggaaacttttgtcggagacggagaagcggccgttcatcgacgaggctaagcggctgcgagcgctgcacatgaaggagcacccggattataaataccggccccggcggaaaaccaagacgctcatgaagaaggataagtacacgctgcccggcgggctgctggcccccggcggcaatagcatggcgagcggggtcggggtgggcgccggcctgggcgcgggcgtgaaccagcgcatggacagttacgcgcacatgaacggctggagcaacggcagctacagcatgatgcaggaccagctgggctacccgcagcacccgggcctcaatgcgcacggcgcagcgcagatgcagcccatgcaccgctacgacgtgagcgccctgcagtacaactccatgaccagctcgcagacctacatgaacggctcgcccacctacagcatgtcctactcgcagcagggcacccctggcatggctcttggctccatgggttcggtggtcaagtccgaggccagctccagcccccctgtggttacctcttcctcccactccagggcgccctgccaggccggggacctccgggacatgatcagcatgtatctccccggcgccgaggtgccggaacccgccgcccccagcagacttcacatgtcccagcactaccagagcggcccggtgcccggcacggccattaacggcacactgcccctctcacacatgacgcgtacgcggccgctcggtaagcctatccctaaccctctcctcggtctcgattctacg

SEQ ID NO: 151 - protein, 330 aa, synthetic construct [sequence omitted]

SEQ ID NO: 152 - DNA, 990 bp, synthetic construct
  source 1..990: mol_type = other DNA
  misc_feature 1..990: note = Fc domain
gcgagcaccaaaggcccgagcgtgtttccgctggcgccgagcagcaaaagcaccagcggcggcaccgcggcgctgggctgcctggtgaaagattattttccggaaccggtgaccgtgagctggaacagcggcgcgctgaccagcggcgtgcatacctttccggcggtgctgcagagcagcggcctgtatagcctgagcagcgtggtgaccgtgccgagcagcagcctgggcacccagacctatatttgcaacgtgaaccataaaccgagcaacaccaaagtggataaaaaagtggaaccgaaaagctgcgataaaacccatacctgcccgccgtgcccggcgccggaactgctgggcggcccgagcgtgtttctgtttccgccgaaaccgaaagataccctgatgattagccgcaccccggaagtgacctgcgtggtggtggatgtgagccatgaagatccggaagtgaaatttaactggtatgtggatggcgtggaagtgcataacgcgaaaaccaaaccgcgcgaagaacagtataacagcacctatcgcgtggtgagcgtgctgaccgtgctgcatcaggattggctgaacggcaaagaatataaatgcaaagtgagcaacaaagcgctgccggcgccgattgaaaaaaccattagcaaagcgaaaggccagccgcgcgaaccgcaggtgtataccctgccgccgagccgcgatgaactgaccaaaaaccaggtgagcctgacctgcctggtgaaaggcttttatccgagcgatattgcggtggaatgggaaagcaacggccagccggaaaacaactataaaaccaccccgccggtgctggatagcgatggcagcttttttctgtatagcaaactgaccgtggataaaagccgctggcagcagggcaacgtgtttagctgcagcgtgatgcatgaagcgctgcataaccattatacccagaaaagcctgagcctgagcccgggcaaa

SEQ ID NO: 153 - protein, 295 aa, synthetic construct
  REGION 1..295: note = halo tag
EIGTGFPFDPHYVEVLGERMHYVDVGPRDGTPVLFLHGNPTSSYVWRNIIPHVAPTHRCIAPDLIGMGKSDKPDLGYFFDDHVRFMDAFIEALGLEEVVLVIHDWGSALGFHWAKRNPERVKGIAFMEFIRPIPTWDEWPEFARETFQAFRTTDVGRKLIIDQNVFIEGTLPMGVVRPLTEVEMDHYREPFLNPVDREPLWRFPNELPIAGEPANIVALVEEYMDWLHQSPVPKLLFWGTPGVLIPPAEAARLAKSLPNCKAVDIGPGLNLLQEDNPDLIGSEIARWLSTLEISG

SEQ ID NO: 154 - DNA, 885 bp, synthetic construct
  source 1..885: mol_type = other DNA
  misc_feature 1..885: note = halo tag
gaaatcggtactggctttccattcgacccccattatgtggaagtcctgggcgagcgcatgcactacgtcgatgttggtccgcgcgatggcacccctgtgctgttcctgcacggtaacccgacctcctcctacgtgtggcgcaacatcatcccgcatgttgcaccgacccatcgctgcattgctccagacctgatcggtatgggcaaatccgacaaaccagacctgggttatttcttcgacgaccacgtccgcttcatggatgccttcatcgaagccctgggtctggaagaggtcgtcctggtcattcacgactggggctccgctctgggtttccactgggccaagcgcaatccagagcgcgtcaaaggtattgcatttatggagttcatccgccctatcccgacctgggacgaatggccagaatttgcccgcgagaccttccaggccttccgcaccaccgacgtcggccgcaagctgatcatcgatcagaacgtttttatcgagggtacgctgccgatgggtgtcgtccgcccgctgactgaagtcgagatggaccattaccgcgagccgttcctgaatcctgttgaccgcgagccactgtggcgcttcccaaacgagctgccaatcgccggtgagccagcgaacatcgtcgcgctggtcgaagaatacatggactggctgcaccagtcccctgtcccgaagctgctgttctggggcaccccaggcgttctgatcccaccggccgaagccgctcgcctggccaaaagcctgcctaactgcaaggctgtggacatcggcccgggtctgaatctgctgcaagaagacaacccggacctgatcggcagcgagatcgcgcgctggctgtctactctggagatttccggt

SEQ ID NO: 155 - protein, 170 aa, synthetic construct
  REGION 1..170: note = NanoLuc tag
VFTLEDFVGDWRQTAGYNLDQVLEQGGVSSLFQNLGVSVTPIQRIVLSGENGLKIDIHVIIPYEGLSGDQMGQIEKIFKVVYPVDDHHFKVILHYGTLVIDGVTPNMIDYFGRPYEGIAVFDGKKITVTGTLWNGNKIIDERLINPDGSLLFRVTINGVTGWRLCERILA

SEQ ID NO: 156 - DNA, 510 bp, synthetic construct
  source 1..510: mol_type = other DNA
  misc_feature 1..510: note = NanoLuc tag
gtcttcacactcgaagatttcgttggggactggcgacagacagccggctacaacctggaccaagtccttgaacagggaggtgtgtccagtttgtttcagaatctcggggtgtccgtaactccgatccaaaggattgtcctgagcggtgaaaatgggctgaagatcgacatccatgtcatcatcccgtatgaaggtctgagcggcgaccaaatgggccagatcgaaaaaatttttaaggtggtgtaccctgtggatgatcatcactttaaggtgatcctgcactatggcacactggtaatcgacggggttacgccgaacatgatcgactatttcggacggccgtatgaaggcatcgccgtgttcgacggcaaaaagatcactgtaacagggaccctgtggaacggcaacaaaattatcgacgagcgcctgatcaaccccgacggctccctgctgttccgagtaaccatcaacggagtgaccggctggcggctgtgcgaacgcattctggcg

SEQ ID NO: 157 - skipped

SEQ ID NO: 158 - protein, 10 aa, synthetic construct
  REGION 1..10: note = myc tag
EQKLISEEDL

SEQ ID NO: 159 - DNA, 30 bp, synthetic construct
  source 1..30: mol_type = other DNA
  misc_feature 1..30: note = myc tag
gagcagaaactcatctcagaagaggatctg

SEQ ID NO: 160 - protein, 14 aa, synthetic construct
  REGION 1..14: note = V5 tag
GKPIPNPLLGLDST

SEQ ID NO: 161 - DNA, 42 bp, synthetic construct
  source 1..42: mol_type = other DNA
  misc_feature 1..42: note = V5 tag
ggtaagcctatccctaaccctctcctcggtctcgattctacg

SEQ ID NO: 162 - protein, 8 aa, synthetic construct
  REGION 1..8: note = flag tag
DYKDDDDK

SEQ ID NO: 163 - DNA, 24 bp, synthetic construct
  source 1..24: mol_type = other DNA
  misc_feature 1..24: note = Flag tag
gactacaaggacgacgatgacaag

SEQ ID NO: 164 - protein, 382 aa, synthetic construct
  REGION 1..382: note = bTrCP190-228.GS.S14
DPAEAVLQEKALKFMNSSEREDCNNGEPPRKIIPEKNSLRQTYNSCARLCLNQETVCLASTAMKTENCVAKTKLANGTSSMIVPKQRKLSASYEKEKELCVKYFEQWSESDQVEFVEHLISQMCHYQHGHINSYLKPMLQRDFITALPARGLDHIAENILSYLDAKSLCAAELVCKEWYRVTSDGMLWKKLIERMVRTDSLWRGLAERRGWGQYLFKNKPPDGNAPPNSFYRALYPKIIQDIETIESNWRCGRHSLQRIHCRGSQVKLEESGGGSVQTGGSLRLTCAASGSIFSMNRMGWFRQAPGKERELVAVIDSKRNKTHYADSVKGRFTISRDNAKNTVDLQMNSLKPEDTAIYYCTAWTGRPPRGYWGQGTQVTVSS

SEQ ID NO: 165 - protein, 295 aa, synthetic construct
  REGION 1..295: note = SKP2 2-176.GS.S14
HRKHLQEIPDLSSNVATSFTWGWDSSKTSELLSGMGVSALEKEEPDSENIPQELLSNLGHPESPPRKRLKSKGSDKDFVIVRRPKLNRENFPGVSWDSLPDELLLGIFSCLCLPELLKVSGVCKRWYRLASDESLWQTLDLTGKNLHPDVTGRLLSQGVIAFRCPRSFMDQPLAEGSQVKLEESGGGSVQTGGSLRLTCAASGSIFSMNRMGWFRQAPGKERELVAVIDSKRNKTHYADSVKGRFTISRDNAKNTVDLQMNSLKPEDTAIYYCTAWTGRPPRGYWGQGTQVTVSS

SEQ ID NO: 166 - protein, 182 aa, synthetic construct
  REGION 1..182: note = S14.GS.VHL152-213
QVKLEESGGGSVQTGGSLRLTCAASGSIFSMNRMGWFRQAPGKERELVAVIDSKRNKTHYADSVKGRFTISRDNAKNTVDLQMNSLKPEDTAIYYCTAWTGRPPRGYWGQGTQVTVSSGSTLPVYTLKERCLQVVRSLVKPENYRRLDIVRSLYEDLEDHPNVQKDLERLTQERIAHQRMGD

SEQ ID NO: 167 - protein, 328 aa, synthetic construct
  REGION 1..328: note = S14.GS.SPOP167-374
QVKLEESGGGSVQTGGSLRLTCAASGSIFSMNRMGWFRQAPGKERELVAVIDSKRNKTHYADSVKGRFTISRDNAKNTVDLQMNSLKPEDTAIYYCTAWTGRPPRGYWGQGTQVTVSSGSSVNISGQNTMNMVKVPECRLADELGGLWENSRFTDCCLCVAGQEFQAHKAILAARSPVFSAMFEHEMEESKKNRVEINDVEPEVFKEMMCFIYTGKAPNLDKMADDLLAAADKYALERLKVMCEDALCSNLSVENAAEILILADLHSADQLKTQAVDFINYHASDVLETSGWKSMVVSHPHLVAEAYRSLASAQCPFLGPPRKRLKQS

SEQ ID NO: 168 - protein, 176 aa, synthetic construct
  REGION 1..176: note = S14.GS.SOCS2 143-198
QVKLEESGGGSVQTGGSLRLTCAASGSIFSMNRMGWFRQAPGKERELVAVIDSKRNKTHYADSVKGRFTISRDNAKNTVDLQMNSLKPEDTAIYYCTAWTGRPPRGYWGQGTQVTVSSGSPRNGTVHLYLTKPLYTSAPSLQHLCRLTINKCTGAIWGLPLPTRLKDYLEEYKFQV

SEQ ID NO: 169 - protein, 296 aa, synthetic construct
  REGION 1..296: note = S14.GS.CHIP128-303
QVKLEESGGGSVQTGGSLRLTCAASGSIFSMNRMGWFRQAPGKERELVAVIDSKRNKTHYADSVKGRFTISRDNAKNTVDLQMNSLKPEDTAIYYCTAWTGRPPRGYWGQGTQVTVSSGSRLNFGDDIPSALRIAKKKRWNSIEERRIHQESELHSYLSRLIAAERERELEECQRNHEGDEDDSHVRAQQACIEAKHDKYMADMDELFSQVDEKRKKRDIPDYLCGKISFELMREPCITPSGITYDRKDIEEHLQRVGHFDPVTRSPLTQEQLIPNLAMKEVIDAFISENGWVEDY

SEQ ID NO: 170 - protein, 233 aa, synthetic construct
  REGION 1..233: note = DDB22-114.GS.S14
APKKRPETQKTSEIVLRPRNKRSRSPLELEPEAKKLCAKGSGPSRRCDSDCLWVGLAGPQILPPCRSIVRTLHQHKLGRASWPSVQQGLQQSFLHTLDSYRILQKAAPFDRRAGSQVKLEESGGGSVQTGGSLRLTCAASGSIFSMNRMGWFRQAPGKERELVAVIDSKRNKTHYADSVKGRFTISRDNAKNTVDLQMNSLKPEDTAIYYCTAWTGRPPRGYWGQGTQVTVSS

SEQ ID NO: 171 - protein, 439 aa, synthetic construct
  REGION 1..439: note = CRBN2-320.GS.S14
AGEGDQQDAAHNMGNHLPLLPAESEEEDEMEVEDQDSKEAKKPNIINFDTSLPTSHTYLGADMEEFHGRTLHDDDSCQVIPVLPQVMMILIPGQTLPLQLFHPQEVSMVRNLIQKDRTFAVLAYSNVQEREAQFGTTAEIYAYREEQDFGIEIVKVKAIGRQRFKVLELRTQSDGIQQAKVQILPECVLPSTMSAVQLESLNKCQIFPSKPVSREDQCSYKWWQKYQKRKFHCANLTSWPRWLYSLYDAETLMDRIKKQLREWDENLKDDSLPSNPIDFSYRVAACLPIDDVLRIQLLKIGSAIQRLRCELDIMNKCTSGSQVKLEESGGGSVQTGGSLRLTCAASGSIFSMNRMGWFRQAPGKERELVAVIDSKRNKTHYADSVKGRFTISRDNAKNTVDLQMNSLKPEDTAIYYCTAWTGRPPRGYWGQGTQVTVSS

SEQ ID NO: 172 - protein, 190 aa, synthetic construct
  REGION 1..190: note = S14.GS.ASB1 266-335
QVKLEESGGGSVQTGGSLRLTCAASGSIFSMNRMGWFRQAPGKERELVAVIDSKRNKTHYADSVKGRFTISRDNAKNTVDLQMNSLKPEDTAIYYCTAWTGRPPRGYWGQGTQVTVSSGSVKWESLGPESRGRRKVDPEALQVFKEARSVPRTLLCLCRVAVRRALGKHRLHLIPSLPLPDPIKKFLLHE

SEQ ID NO: 173 - protein, 204 aa, synthetic construct
  REGION 1..204: note = TRIM21 2-85.GS.S14
ASAARLTMMWEEVTCPICLDPFVEPVSIECGHSFCQECISQVGKGGGSVCPVCRQRFLLKNLRPNRQLANMVNNLKEISQEAREGSQVKLEESGGGSVQTGGSLRLTCAASGSIFSMNRMGWFRQAPGKERELVAVIDSKRNKTHYADSVKGRFTISRDNAKNTVDLQMNSLKPEDTAIYYCTAWTGRPPRGYWGQGTQVTVSS

SEQ ID NO: 174 - protein, 240 aa, synthetic construct
  REGION 1..240: note = S14.GS.RNF4 71-190
QVKLEESGGGSVQTGGSLRLTCAASGSIFSMNRMGWFRQAPGKERELVAVIDSKRNKTHYADSVKGRFTISRDNAKNTVDLQMNSLKPEDTAIYYCTAWTGRPPRGYWGQGTQVTVSSGSDERRRPRRNARRLPQDHADSCVVSSDDEELSRDRDVYVTTHTPRNARDEGATGLRPSGTVSCPICMDGYSEIVQNGRLIVSTECGHVFCSQCLRDSLKNANTCPTCRKKINHKRYHPIYI

SEQ ID NO: 175 - protein, 190 aa, synthetic construct
  REGION 1..190: note = 3A2.GS.VHL152-213
EVQLVESGGEQVQPGSSLKLSCSVSGLMISGHAMSWVRQVPGAGPEWVAVDNPGGKKNYIDSVAGRFTIARDNDANSLSLVMNGLRPEDTARYFCARVLSFKIYEGDKWALEWDYRGPGTQVTVSSGSTLPVYTLKERCLQVVRSLVKPENYRRLDIVRSLYEDLEDHPNVQKDLERLTQERIAHQRMGD

SEQ ID NO: 176 - protein, 336 aa, synthetic construct
  REGION 1..336: note = 3A2.GS.SPOP167-374
EVQLVESGGEQVQPGSSLKLSCSVSGLMISGHAMSWVRQVPGAGPEWVAVDNPGGKKNYIDSVAGRFTIARDNDANSLSLVMNGLRPEDTARYFCARVLSFKIYEGDKWALEWDYRGPGTQVTVSSGSSVNISGQNTMNMVKVPECRLADELGGLWENSRFTDCCLCVAGQEFQAHKAILAARSPVFSAMFEHEMEESKKNRVEINDVEPEVFKEMMCFIYTGKAPNLDKMADDLLAAADKYALERLKVMCEDALCSNLSVENAAEILILADLHSADQLKTQAVDFINYHASDVLETSGWKSMVVSHPHLVAEAYRSLASAQCPFLGPPRKRLKQS

SEQ ID NO: 177 - protein, 184 aa, synthetic construct
  REGION 1..184: note = 3A2.GS.SOCS2 143-198
EVQLVESGGEQVQPGSSLKLSCSVSGLMISGHAMSWVRQVPGAGPEWVAVDNPGGKKNYIDSVAGRFTIARDNDANSLSLVMNGLRPEDTARYFCARVLSFKIYEGDKWALEWDYRGPGTQVTVSSGSPRNGTVHLYLTKPLYTSAPSLQHLCRLTINKCTGAIWGLPLPTRLKDYLEEYKFQV

SEQ ID NO: 178 - protein, 304 aa, synthetic construct
  REGION 1..304: note = 3A2.GS.CHIP128-303
EVQLVESGGEQVQPGSSLKLSCSVSGLMISGHAMSWVRQVPGAGPEWVAVDNPGGKKNYIDSVAGRFTIARDNDANSLSLVMNGLRPEDTARYFCARVLSFKIYEGDKWALEWDYRGPGTQVTVSSGSRLNFGDDIPSALRIAKKKRWNSIEERRIHQESELHSYLSRLIAAERERELEECQRNHEGDEDDSHVRAQQACIEAKHDKYMADMDELFSQVDEKRKKRDIPDYLCGKISFELMREPCITPSGITYDRKDIEEHLQRVGHFDPVTRSPLTQEQLIPNLAMKEVIDAFISENGWVEDY

SEQ ID NO: 179 - protein, 198 aa, synthetic construct
  REGION 1..198: note = 3A2GS.ASB1 266-335
EVQLVESGGEQVQPGSSLKLSCSVSGLMISGHAMSWVRQVPGAGPEWVAVDNPGGKKNYIDSVAGRFTIARDNDANSLSLVMNGLRPEDTARYFCARVLSFKIYEGDKWALEWDYRGPGTQVTVSSGSVKWESLGPESRGRRKVDPEALQVFKEARSVPRTLLCLCRVAVRRALGKHRLHLIPSLPLPDPIKKFLLHE

SEQ ID NO: 180 - protein, 212 aa, synthetic construct
  REGION 1..212: note = TRIM21 2-85.GS.3A2
ASAARLTMMWEEVTCPICLDPFVEPVSIECGHSFCQECISQVGKGGGSVCPVCRQRFLLKNLRPNRQLANMVNNLKEISQEAREGSEVQLVESGGEQVQPGSSLKLSCSVSGLMISGHAMSWVRQVPGAGPEWVAVDNPGGKKNYIDSVAGRFTIARDNDANSLSLVMNGLRPEDTARYFCARVLSFKIYEGDKWALEWDYRGPGTQVTVSS

SEQ ID NO: 181 - protein, 248 aa, synthetic construct
  REGION 1..248: note = 3A2.GS.RNF4 71-190
EVQLVESGGEQVQPGSSLKLSCSVSGLMISGHAMSWVRQVPGAGPEWVAVDNPGGKKNYIDSVAGRFTIARDNDANSLSLVMNGLRPEDTARYFCARVLSFKIYEGDKWALEWDYRGPGTQVTVSSGSDERRRPRRNARRLPQDHADSCVVSSDDEELSRDRDVYVTTHTPRNARDEGATGLRPSGTVSCPICMDGYSEIVQNGRLIVSTECGHVFCSQCLRDSLKNANTCPTCRKKINHKRYHPIYI

SEQ ID NO: 182 - protein, 274 aa, synthetic construct
  REGION 1..274: note = 3A2.GS.UBE2D1 2-147
EVQLVESGGEQVQPGSSLKLSCSVSGLMISGHAMSWVRQVPGAGPEWVAVDNPGGKKNYIDSVAGRFTIARDNDANSLSLVMNGLRPEDTARYFCARVLSFKIYEGDKWALEWDYRGPGTQVTVSSGSALKRIQKELSDLQRDPPAHCSAGPVGDDLFHWQATIMGPPDSAYQGGVFFLTVHFPTDYPFKPPKIAFTTKIYHPNINSNGSICLDILRSQWSPALTVSKVLLSICSLLCDPNPDDPLVPDIAQIYKSDKEKYNRHAREWTQKYAM

SEQ ID NO: 183 - protein, 274 aa, synthetic construct
  REGION 1..274: note = 3A2.GS.UBE2D4 2-147
EVQLVESGGEQVQPGSSLKLSCSVSGLMISGHAMSWVRQVPGAGPEWVAVDNPGGKKNYIDSVAGRFTIARDNDANSLSLVMNGLRPEDTARYFCARVLSFKIYEGDKWALEWDYRGPGTQVTVSSGSALKRIQKELTDLQRDPPAQCSAGPVGDDLFHWQATIMGPNDSPYQGGVFFLTIHFPTDYPFKPPKVAFTTKIYHPNINSNGSICLDILRSQWSPALTVSKVLLSICSLLCDPNPDDPLVPEIAHTYKADREKYNRLAREWTQKYAM

SEQ ID NO: 184 - protein, 218 aa, synthetic construct
  REGION 1..218: note = 3A2.GS.ZNFR1 138-227
EVQLVESGGEQVQPGSSLKLSCSVSGLMISGHAMSWVRQVPGAGPEWVAVDNPGGKKNYIDSVAGRFTIARDNDANSLSLVMNGLRPEDTARYFCARVLSFKIYEGDKWALEWDYRGPGTQVTVSSGSSSHSGFKCPICSKSVASDEMEMHFIMCLSKPRLSYNDDVLTKDAGECVICLEELLQGDTIARLPCLCIYHKSCIDSWFEVNRSCPEHPAD

SEQ ID NO: 185 - DNA, 1146 bp, synthetic construct
  source 1..1146: mol_type = other DNA
  misc_feature 1..1146: note = bTrCP190-228.GS.S14
gacccggccgaggcggtgctgcaagagaaggcactcaagtttatgaactcctcagagagagaagactgtaataatggcgaaccccctaggaagataataccagagaagaactcacttagacagacatacaacagctgtgccagactctgcttaaaccaagaaacagtatgtttagcaagcactgctatgaagactgagaattgtgtggccaaaacaaaacttgccaatggcacttccagtatgattgtgcccaagcaacggaaactctcagcaagctatgaaaaggaaaaggaactgtgtgtcaaatactttgagcagtggtcagagtcagatcaagtggaatttgtggaacatcttatatcccaaatgtgtcattaccaacatgggcacataaactcgtatcttaaacctatgttgcagagagatttcataactgctctgccagctcggggattggatcatattgctgagaacattctgtcatacctggatgccaaatcactatgtgctgctgaacttgtgtgcaaggaatggtaccgagtgacctctgatggcatgctgtggaagaagcttatcgagagaatggtcaggacagattctctgtggagaggcctggcagaacgaagaggatggggacagtatttattcaaaaacaaacctcctgacgggaatgctcctcccaactctttttatagagcactttatcctaaaattatacaagacattgagacaatagaatctaattggagatgtggaagacatagtttacagaggattcactgccgaggatcccaggtgaagctggaggagagcggcggcggcagcgtgcagaccggcggcagcctgaggctgacctgcgccgccagcggcagcatcttcagcatgaacaggatgggctggttcaggcaggcccccggcaaggagagggagctggtggccgtgatcgacagcaagaggaacaagacccactacgccgacagcgtgaagggcaggttcaccatcagcagggacaacgccaagaacaccgtggacctccagatgaacagcctgaagcccgaggacaccgccatctactactgcaccgcctggaccggcaggccccccaggggctactggggccagggcacccaggtgaccgtgagcagc

SEQ ID NO: 186 - DNA, 885 bp, synthetic construct
  source 1..885: mol_type = other DNA
  misc_feature 1..885: note = SKP22-176.GS.S14
cacaggaagcacctccaggagattccagacctgagtagcaacgttgccaccagcttcacgtggggatgggattccagcaagacttctgaactgctgtcaggcatgggggtctccgccctggagaaagaggagcccgacagtgagaacatcccccaggaactgctctcaaacctgggccacccggagagccccccacggaaacggctgaagagcaaagggagtgacaaagactttgtgattgtccgcaggcctaagctaaatcgagagaactttccaggtgtttcatgggactcccttccggatgagctgctcttgggaatcttttcctgtctgtgcctccctgagctgctaaaggtctctggtgtttgtaagaggtggtatcgcctagcgtctgatgagtctctatggcagaccttagacctcacaggtaaaaatctgcacccggatgtgactggtcggttgctgtctcaaggggtgattgccttccgctgcccacgatcatttatggaccaaccattggctgaaggatcccaggtgaagctggaggagagcggcggcggcagcgtgcagaccggcggcagcctgaggctgacctgcgccgccagcggcagcatcttcagcatgaacaggatgggctggttcaggcaggcccccggcaaggagagggagctggtggccgtgatcgacagcaagaggaacaagacccactacgccgacagcgtgaagggcaggttcaccatcagcagggacaacgccaagaacaccgtggacctccagatgaacagcctgaagcccgaggacaccgccatctactactgcaccgcctggaccggcaggccccccaggggctactggggccagggcacccaggtgaccgtgagcagc

SEQ ID NO: 187 - DNA, 546 bp, synthetic construct
  source 1..546: mol_type = other DNA
  misc_feature 1..546: note = S14.GS.VHL152-213
caggtgaagctggaggagagcggcggcggcagcgtgcagaccggcggcagcctgaggctgacctgcgccgccagcggcagcatcttcagcatgaacaggatgggctggttcaggcaggcccccggcaaggagagggagctggtggccgtgatcgacagcaagaggaacaagacccactacgccgacagcgtgaagggcaggttcaccatcagcagggacaacgccaagaacaccgtggacctccagatgaacagcctgaagcccgaggacaccgccatctactactgcaccgcctggaccggcaggccccccaggggctactggggccagggcacccaggtgaccgtgagcagcggatccacactgccagtgtatactctgaaagagcgatgcctccaggttgtccggagcctagtcaagcctgagaattacaggagactggacatcgtcaggtcgctctacgaagatctggaagaccacccaaatgtgcagaaagacctggagcggctgacacaggagcgcattgcacatcaacggatgggagat

SEQ ID NO: 188 - DNA, 984 bp, synthetic construct
  source 1..984: mol_type = other DNA
  misc_feature 1..984: note = S14.GS.SPOP167-374
caggtgaagctggaggagagcggcggcggcagcgtgcagaccggcggcagcctgaggctgacctgcgccgccagcggcagcatcttcagcatgaacaggatgggctggttcaggcaggcccccggcaaggagagggagctggtggccgtgatcgacagcaagaggaacaagacccactacgccgacagcgtgaagggcaggttcaccatcagcagggacaacgccaagaacaccgtggacctccagatgaacagcctgaagcccgaggacaccgccatctactactgcaccgcctggaccggcaggccccccaggggctactggggccagggcacccaggtgaccgtgagcagcggatcctctgtcaacatttctggccagaataccatgaacatggtaaaggttcctgagtgccggctggcagatgagttaggaggactgtgggagaactcccggttcacagactgctgcttgtgtgttgccggccaggagttccaggctcacaaggctatcttagcagctcgttctccggtttttagtgccatgtttgaacatgaaatggaggagagcaaaaagaatcgagttgaaatcaatgatgtggagcctgaagtttttaaggaaatgatgtgcttcatttacacggggaaggctccaaacctcgacaaaatggctgatgatttgctggcagctgctgacaagtatgccctggagcgcttaaaggtcatgtgtgaggatgccctctgtagtaacctgtccgtggagaacgcagctgaaattctcatcctggccgacctccacagtgcagatcagttgaaaactcaggcagtggatttcatcaactatcatgcttcggatgtcttggagacctctgggtggaagtcaatggtggtgtcacatccccacttggtggctgaggcataccgctctctggcttcagcacagtgcccttttctgggacccccacgcaaacgcctgaagcaatcc

SEQ ID NO: 189 - DNA, 528 bp, synthetic construct
  source 1..528: mol_type = other DNA
  misc_feature 1..528: note = S14.GS.SOCS2 143-198
caggtgaagctggaggagagcggcggcggcagcgtgcagaccggcggcagcctgaggctgacctgcgccgccagcggcagcatcttcagcatgaacaggatgggctggttcaggcaggcccccggcaaggagagggagctggtggccgtgatcgacagcaagaggaacaagacccactacgccgacagcgtgaagggcaggttcaccatcagcagggacaacgccaagaacaccgtggacctccagatgaacagcctgaagcccgaggacaccgccatctactactgcaccgcctggaccggcaggccccccaggggctactggggccagggcacccaggtgaccgtgagcagcggatccccccggaacggcactgttcacctttatctgaccaaaccgctctacacgtcagcaccatctctccagcatctctgtaggctcaccattaacaaatgtaccggtgccatctggggactgcctttaccaacaagactaaaagattacttggaagaatataaattccaggta

SEQ ID NO: 190 - DNA, 888 bp, synthetic construct
  source 1..888: mol_type = other DNA
  misc_feature 1..888: note = S14.GS.CHIP 128-303
caggtgaagctggaggagagcggcggcggcagcgtgcagaccggcggcagcctgaggctgacctgcgccgccagcggcagcatcttcagcatgaacaggatgggctggttcaggcaggcccccggcaaggagagggagctggtggccgtgatcgacagcaagaggaacaagacccactacgccgacagcgtgaagggcaggttcaccatcagcagggacaacgccaagaacaccgtggacctccagatgaacagcctgaagcccgaggacaccgccatctactactgcaccgcctggaccggcaggccccccaggggctactggggccagggcacccaggtgaccgtgagcagcggatcccggctgaacttcggggacgacatccccagcgctcttcgaatcgcgaagaagaagcgctggaacagcattgaggagcggcgcatccaccaggagagcgagctgcactcctacctctccaggctcattgccgcggagcgtgagagggagctggaagagtgccagcgaaaccacgagggtgatgaggacgacagccacgtccgggcccagcaggcctgcattgaggccaagcacgacaagtacatggcggacatggacgagcttttttctcaggtggatgagaagaggaagaagcgagacatccccgactacctgtgtggcaagatcagctttgagctgatgcgggagccgtgcatcacgcccagtggcatcacctacgaccgcaaggacatcgaggagcacctccagcgtgtgggtcattttgaccccgtgacccggagccccctgacccaggaacagctcatccccaacttggctatgaaggaggttattgacgcattcatctctgagaatggctgggtggaggactac

SEQ ID NO: 191 - DNA, 699 bp, synthetic construct
  source 1..699: mol_type = other DNA
  misc_feature 1..699: note = DDB2 2-114.GS.S14
gctcccaagaaacgcccagaaacccagaagacctccgagattgtattacgccccaggaacaagaggagcaggagtcccctggagctggagcccgaggccaagaagctctgtgcgaagggctccggtcctagcagaagatgtgactcagactgcctctgggtggggctggctggcccacagatcctgccaccatgccgcagcatcgtcaggaccctccaccagcataagctgggcagagcttcctggccatctgtccagcaggggctccagcagtcctttttgcacactctggattcttaccggatattacaaaaggctgccccctttgacaggagggctggatcccaggtgaagctggaggagagcggcggcggcagcgtgcagaccggcggcagcctgaggctgacctgcgccgccagcggcagcatcttcagcatgaacaggatgggctggttcaggcaggcccccggcaaggagagggagctggtggccgtgatcgacagcaagaggaacaagacccactacgccgacagcgtgaagggcaggttcaccatcagcagggacaacgccaagaacaccgtggacctccagatgaacagcctgaagcccgaggacaccgccatctactactgcaccgcctggaccggcaggccccccaggggctactggggccagggcacccaggtgaccgtgagcagc

SEQ ID NO: 192 - DNA, 1317 bp, synthetic construct
  source 1..1317: mol_type = other DNA
  misc_feature 1..1317: note = CRBN2-320.GS.S14
gccggcgaaggagatcagcaggacgctgcgcacaacatgggcaaccacctgccgctcctgccagcagagagtgaggaagaagatgaaatggaagttgaagaccaggatagtaaagaagccaaaaaaccaaacatcataaattttgacaccagtctgccgacatcacatacatacctaggtgctgatatggaagaatttcatggcaggactttgcacgatgacgacagctgtcaggtgattccagttcttccacaagtgatgatgatcctgattcccggacagacattacctcttcagctttttcaccctcaagaagtcagtatggtgcggaatttaattcagaaagatagaacctttgctgttcttgcatacagcaatgtacaggaaagggaagcacagtttggaacaacagcagagatatatgcctatcgagaagaacaggattttggaattgagatagtgaaagtgaaagcaattggaagacaaaggttcaaagtccttgagctaagaacacagtcagatggaatccagcaagctaaagtgcaaattcttcccgaatgtgtgttgccttcaaccatgtcagcagttcaattagaatccctcaataagtgccagatatttccttcaaaacctgtctcaagagaagaccaatgttcatataaatggtggcagaaataccagaagagaaagtttcattgtgcaaatctaacttcatggcctcgctggctgtattccttatatgatgctgagaccttaatggacagaatcaagaaacagctacgtgaatgggatgaaaatctaaaagatgattctcttccttcaaatccaatagatttttcttacagagtagctgcttgtcttcctattgatgatgtattgagaatacagctccttaaaattggcagtgctatccagcgacttcgctgtgaattagacattatgaataaatgtacttccggatcccaggtgaagctggaggagagcggcggcggcagcgtgcagaccggcggcagcctgaggctgacctgcgccgccagcggcagcatcttcagcatgaacaggatgggctggttcaggcaggcccccggcaaggagagggagctggtggccgtgatcgacagcaagaggaacaagacccactacgccgacagcgtgaagggcaggttcaccatcagcagggacaacgccaagaacaccgtggacctccagatgaacagcctgaagcccgaggacaccgccatctactactgcaccgcctggaccggcaggccccccaggggctactggggccagggcacccaggtgaccgtgagcagc

SEQ ID NO: 193 - DNA, 570 bp, synthetic construct
  source 1..570: mol_type = other DNA
  misc_feature 1..570: note = S14.GS.ASB1 266-335
caggtgaagctggaggagagcggcggcggcagcgtgcagaccggcggcagcctgaggctgacctgcgccgccagcggcagcatcttcagcatgaacaggatgggctggttcaggcaggcccccggcaaggagagggagctggtggccgtgatcgacagcaagaggaacaagacccactacgccgacagcgtgaagggcaggttcaccatcagcagggacaacgccaagaacaccgtggacctccagatgaacagcctgaagcccgaggacaccgccatctactactgcaccgcctggaccggcaggccccccaggggctactggggccagggcacccaggtgaccgtgagcagcggatccgtgaagtgggaatcgctgggcccagagtcgagaggaagaagaaaagtggaccctgaggccttgcaggtctttaaagaggccagaagtgttcccagaaccttgctgtgtctgtgccgtgtggctgtgagaagagctcttggcaaacaccggcttcatctgattccttcgctgcctctgccagaccccataaagaagtttctactccatgag

SEQ ID NO: 194 - DNA, 612 bp, synthetic construct
  source 1..612: mol_type = other DNA
  misc_feature 1..612: note = TRIM21 2-85.GS.S14
gcttcagcagcacgcttgacaatgatgtgggaggaggtcacatgccctatctgcctggaccccttcgtggagcctgtgagcatcgagtgtggccacagcttctgccaggaatgcatctctcaggttgggaaaggtgggggcagcgtctgtcctgtgtgccggcagcgctttctgctcaagaatctccggcccaatcgacagctagccaacatggtgaacaaccttaaagaaatcagccaggaggccagagagggatcccaggtgaagctggaggagagcggcggcggcagcgtgcagaccggcggcagcctgaggctgacctgcgccgccagcggcagcatcttcagcatgaacaggatgggctggttcaggcaggcccccggcaaggagagggagctggtggccgtgatcgacagcaagaggaacaagacccactacgccgacagcgtgaagggcaggttcaccatcagcagggacaacgccaagaacaccgtggacctccagatgaacagcctgaagcccgaggacaccgccatctactactgcaccgcctggaccggcaggccccccaggggctactggggccagggcacccaggtgaccgtgagcagc

SEQ ID NO: 195 - DNA, 720 bp, synthetic construct
  source 1..720: mol_type = other DNA
  misc_feature 1..720: note = S14.GS.RNF4 71-190
caggtgaagctggaggagagcggcggcggcagcgtgcagaccggcggcagcctgaggctgacctgcgccgccagcggcagcatcttcagcatgaacaggatgggctggttcaggcaggcccccggcaaggagagggagctggtggccgtgatcgacagcaagaggaacaagacccactacgccgacagcgtgaagggcaggttcaccatcagcagggacaacgccaagaacaccgtggacctccagatgaacagcctgaagcccgaggacaccgccatctactactgcaccgcctggaccggcaggccccccaggggctactggggccagggcacccaggtgaccgtgagcagcggatccgacgaaagaagaagaccaaggaggaatgctaggaggctgccccaggaccatgctgacagctgtgtggtgagcagtgacgatgaggagttgtccagggacagagacgtatatgtgactacccatactcccagaaacgccagggatgagggcgctacaggcctcaggccctcaggtactgtcagttgtcccatctgcatggacggatactcagagatcgtgcagaatggacgtctcatcgtttccacagaatgcggccatgtcttctgtagccagtgcctccgtgattccctgaagaatgctaatacttgcccaacttgtaggaaaaagatcaaccacaaacggtaccaccccatttatata

SEQ ID NO: 196 - DNA, 570 bp, synthetic construct
  source 1..570: mol_type = other DNA
  misc_feature 1..570: note = 3A2.GS.VHL152-213
gaggtgcaattggttgagtcaggaggtgagcaggtccaacctggtagttctttgaaattgagctgttcagtctcaggtctgatgatatcaggccacgcgatgagttgggtcaggcaagtaccgggggccgggcctgagtgggtcgcggtggataatccagggggtaaaaagaactatattgactcagttgctggcagatttacgattgctcgggacaacgatgcaaactctctgagcctcgttatgaacggtctgcggcctgaggacacagccaggtacttctgcgcccgagtattgagctttaagatatacgaaggagataaatgggctctggagtgggactatcgcgggccgggcacacaagtgacggtgtccagcggatccacactgccagtgtatactctgaaagagcgatgcctccaggttgtccggagcctagtcaagcctgagaattacaggagactggacatcgtcaggtcgctctacgaagatctggaagaccacccaaatgtgcagaaagacctggagcggctgacacaggagcgcattgcacatcaacggatgggagat

SEQ ID NO: 197 - DNA, 1008 bp, synthetic construct
  source 1..1008: mol_type = other DNA
  misc_feature 1..1008: note = 3A2.GS.SPOP 167-374
gaggtgcaattggttgagtcaggaggtgagcaggtccaacctggtagttctttgaaattgagctgttcagtctcaggtctgatgatatcaggccacgcgatgagttgggtcaggcaagtaccgggggccgggcctgagtgggtcgcggtggataatccagggggtaaaaagaactatattgactcagttgctggcagatttacgattgctcgggacaacgatgcaaactctctgagcctcgttatgaacggtctgcggcctgaggacacagccaggtacttctgcgcccgagtattgagctttaagatatacgaaggagataaatgggctctggagtgggactatcgcgggccgggcacacaagtgacggtgtccagcggatcctctgtcaacatttctggccagaataccatgaacatggtaaaggttcctgagtgccggctggcagatgagttaggaggactgtgggagaactcccggttcacagactgctgcttgtgtgttgccggccaggagttccaggctcacaaggctatcttagcagctcgttctccggtttttagtgccatgtttgaacatgaaatggaggagagcaaaaagaatcgagttgaaatcaatgatgtggagcctgaagtttttaaggaaatgatgtgcttcatttacacggggaaggctccaaacctcgacaaaatggctgatgatttgctggcagctgctgacaagtatgccctggagcgcttaaaggtcatgtgtgaggatgccctctgtagtaacctgtccgtggagaacgcagctgaaattctcatcctggccgacctccacagtgcagatcagttgaaaactcaggcagtggatttcatcaactatcatgcttcggatgtcttggagacctctgggtggaagtcaatggtggtgtcacatccccacttggtggctgaggcataccgctctctggcttcagcacagtgcccttttctgggacccccacgcaaacgcctgaagcaatcc

SEQ ID NO: 198 - DNA, 552 bp, synthetic construct
  source 1..552: mol_type = other DNA
  misc_feature 1..552: note = 3A2.GS.SOCS2 143-198
gaggtgcaattggttgagtcaggaggtgagcaggtccaacctggtagttctttgaaattgagctgttcagtctcaggtctgatgatatcaggccacgcgatgagttgggtcaggcaagtaccgggggccgggcctgagtgggtcgcggtggataatccagggggtaaaaagaactatattgactcagttgctggcagatttacgattgctcgggacaacgatgcaaactctctgagcctcgttatgaacggtctgcggcctgaggacacagccaggtacttctgcgcccgagtattgagctttaagatatacgaaggagataaatgggctctggagtgggactatcgcgggccgggcacacaagtgacggtgtccagcggatccccccggaacggcactgttcacctttatctgaccaaaccgctctacacgtcagcaccatctctccagcatctctgtaggctcaccattaacaaatgtaccggtgccatctggggactgcctttaccaacaagactaaaagattacttggaagaatataaattccaggta

SEQ ID NO: 199 - DNA, 912 bp, synthetic construct
  source 1..912: mol_type = other DNA
  misc_feature 1..912: note = 3A2.GS.CHIP128-303
gaggtgcaattggttgagtcaggaggtgagcaggtccaacctggtagttctttgaaattgagctgttcagtctcaggtctgatgatatcaggccacgcgatgagttgggtcaggcaagtaccgggggccgggcctgagtgggtcgcggtggataatccagggggtaaaaagaactatattgactcagttgctggcagatttacgattgctcgggacaacgatgcaaactctctgagcctcgttatgaacggtctgcggcctgaggacacagccaggtacttctgcgcccgagtattgagctttaagatatacgaaggagataaatgggctctggagtgggactatcgcgggccgggcacacaagtgacggtgtccagcggatcccggctgaacttcggggacgacatccccagcgctcttcgaatcgcgaagaagaagcgctggaacagcattgaggagcggcgcatccaccaggagagcgagctgcactcctacctctccaggctcattgccgcggagcgtgagagggagctggaagagtgccagcgaaaccacgagggtgatgaggacgacagccacgtccgggcccagcaggcctgcattgaggccaagcacgacaagtacatggcggacatggacgagcttttttctcaggtggatgagaagaggaagaagcgagacatccccgactacctgtgtggcaagatcagctttgagctgatgcgggagccgtgcatcacgcccagtggcatcacctacgaccgcaaggacatcgaggagcacctccagcgtgtgggtcattttgaccccgtgacccggagccccctgacccaggaacagctcatccccaacttggctatgaaggaggttattgacgcattcatctctgagaatggctgggtggaggactac

SEQ ID NO: 200 - DNA, 594 bp, synthetic construct
  source 1..594: mol_type = other DNA
  misc_feature 1..594: note = 3A2GS.ASB1 266-335
gaggtgcaattggttgagtcaggaggtgagcaggtccaacctggtagttctttgaaattgagctgttcagtctcaggtctgatgatatcaggccacgcgatgagttgggtcaggcaagtaccgggggccgggcctgagtgggtcgcggtggataatccagggggtaaaaagaactatattgactcagttgctggcagatttacgattgctcgggacaacgatgcaaactctctgagcctcgttatgaacggtctgcggcctgaggacacagccaggtacttctgcgcccgagtattgagctttaagatatacgaaggagataaatgggctctggagtgggactatcgcgggccgggcacacaagtgacggtgtccagcggatccgtgaagtgggaatcgctgggcccagagtcgagaggaagaagaaaagtggaccctgaggccttgcaggtctttaaagaggccagaagtgttcccagaaccttgctgtgtctgtgccgtgtggctgtgagaagagctcttggcaaacaccggcttcatctgattccttcgctgcctctgccagaccccataaagaagtttctactccatgag

SEQ ID NO: 201 - DNA, 636 bp, synthetic construct
  source 1..636: mol_type = other DNA
  misc_feature 1..636: note = TRIM21 2-85.GS.3A2
gcttcagcagcacgcttgacaatgatgtgggaggaggtcacatgccctatctgcctggaccccttcgtggagcctgtgagcatcgagtgtggccacagcttctgccaggaatgcatctctcaggttgggaaaggtgggggcagcgtctgtcctgtgtgccggcagcgctttctgctcaagaatctccggcccaatcgacagctagccaacatggtgaacaaccttaaagaaatcagccaggaggccagagagggatccgaggtgcaattggttgagtcaggaggtgagcaggtccaacctggtagttctttgaaattgagctgttcagtctcaggtctgatgatatcaggccacgcgatgagttgggtcaggcaagtaccgggggccgggcctgagtgggtcgcggtggataatccagggggtaaaaagaactatattgactcagttgctggcagatttacgattgctcgggacaacgatgcaaactctctgagcctcgttatgaacggtctgcggcctgaggacacagccaggtacttctgcgcccgagtattgagctttaagatatacgaaggagataaatgggctctggagtgggactatcgcgggccgggcacacaagtgacggtgtccagc

SEQ ID NO: 202 - DNA, 744 bp, synthetic construct
  source 1..744: mol_type = other DNA
  misc_feature 1..744: note = 3A2.GS.RNF4 71-190
gaggtgcaattggttgagtcaggaggtgagcaggtccaacctggtagttctttgaaattgagctgttcagtctcaggtctgatgatatcaggccacgcgatgagttgggtcaggcaagtaccgggggccgggcctgagtgggtcgcggtggataatccagggggtaaaaagaactatattgactcagttgctggcagatttacgattgctcgggacaacgatgcaaactctctgagcctcgttatgaacggtctgcggcctgaggacacagccaggtacttctgcgcccgagtattgagctttaagatatacgaaggagataaatgggctctggagtgggactatcgcgggccgggcacacaagtgacggtgtccagcggatccgacgaaagaagaagaccaaggaggaatgctaggaggctgccccaggaccatgctgacagctgtgtggtgagcagtgacgatgaggagttgtccagggacagagacgtatatgtgactacccatactcccagaaacgccagggatgagggcgctacaggcctcaggccctcaggtactgtcagttgtcccatctgcatggacggatactcagagatcgtgcagaatggacgtctcatcgtttccacagaatgcggccatgtcttctgtagccagtgcctccgtgattccctgaagaatgctaatacttgcccaacttgtaggaaaaagatcaaccacaaacggtaccaccccatttatata

SEQ ID NO: 203 - DNA, 822 bp, synthetic construct
  source 1..822: mol_type = other DNA
  misc_feature 1..822: note = 3A2.GS.UBE2D1 2-147
gaggtgcaattggttgagtcaggaggtgagcaggtccaacctggtagttctttgaaattgagctgttcagtctcaggtctgatgatatcaggccacgcgatgagttgggtcaggcaagtaccgggggccgggcctgagtgggtcgcggtggataatccagggggtaaaaagaactatattgactcagttgctggcagatttacgattgctcgggacaacgatgcaaactctctgagcctcgttatgaacggtctgcggcctgaggacacagccaggtacttctgcgcccgagtattgagctttaagatatacgaaggagataaatgggctctggagtgggactatcgcgggccgggcacacaagtgacggtgtccagcggatccgccttgaagcgcatacaaaaagagctctctgaccttcaaagagacccaccagctcactgtagtgcaggtcccgtaggcgacgatctttttcactggcaggcgacgatcatgggcccaccagattccgcttaccagggcggggtttttttcctgaccgttcactttccaactgactatccatttaaacctccgaagatcgcattcacaaccaagatttatcatccgaatatcaatagtaatgggtctatctgtttggacatcctgcgaagccagtggtcccccgcgctgactgtcagtaaagttttgctctctatctgttcccttctgtgcgatccgaacccggacgaccctcttgtcccagacatcgcccagatatacaagtcagataaagaaaaatataatagacacgcccgcgaatggacgcagaagtatgcaatg

SEQ ID NO: 204 - DNA, 822 bp, synthetic construct
  source 1..822: mol_type = other DNA
  misc_feature 1..822: note = 3A2.GS.UBE2D4 2-147
gaggtgcaattggttgagtcaggaggtgagcaggtccaacctggtagttctttgaaattgagctgttcagtctcaggtctgatgatatcaggccacgcgatgagttgggtcaggcaagtaccgggggccgggcctgagtgggtcgcggtggataatccagggggtaaaaagaactatattgactcagttgctggcagatttacgattgctcgggacaacgatgcaaactctctgagcctcgttatgaacggtctgcggcctgaggacacagccaggtacttctgcgcccgagtattgagctttaagatatacgaaggagataaatgggctctggagtgggactatcgcgggccgggcacacaagtgacggtgtccagcggatccgccctgaagcgcatccagaaggaattgactgatcttcagagggacccaccagcgcagtgctcagccggtccggtaggggacgaccttttccactggcaggccacaataatgggtccaaatgactctccataccaagggggtgtgtttttcctcaccatccatttcccgacagactatccattcaagccacctaaagtggctttcacgacaaaaatataccaccccaacattaacagcaacgggagcatttgtttggatatacttagatctcaatggagccccgcactgacggtgagtaaagtccttctgtccatttgtagccttttgtgtgacccgaaccctgatgacccacttgtaccagagattgcgcacacttacaaagcggatagagagaagtataaccgacttgcgagggagtggacgcaaaagtacgccatg

SEQ ID NO: 205 - DNA, 654 bp, synthetic construct
  source 1..654: mol_type = other DNA
  misc_feature 1..654: note = 3A2.GS.ZNFR1 138-227
gaggtgcaattggttgagtcaggaggtgagcaggtccaacctggtagttctttgaaattgagctgttcagtctcaggtctgatgatatcaggccacgcgatgagttgggtcaggcaagtaccgggggccgggcctgagtgggtcgcggtggataatccagggggtaaaaagaactatattgactcagttgctggcagatttacgattgctcgggacaacgatgcaaactctctgagcctcgttatgaacggtctgcggcctgaggacacagccaggtacttctgcgcccgagtattgagctttaagatatacgaaggagataaatgggctctggagtgggactatcgcgggccgggcacacaagtgacggtgtccagcggatccagctcgcatagtggtttcaagtgccccatttgctccaagtctgtggcttctgacgagatggaaatgcactttataatgtgtttgagcaaacctcgcctctcctacaacgatgatgtgctgactaaagacgcgggtgagtgtgtgatctgcctggaggagctgctgcagggggacacgatagccaggctgccctgcctgtgcatctatcacaaaagctgcatagactcgtggtttgaagtgaacagatcttgtccggaacaccctgcggac

SEQ ID NO: 206 - protein, 262 aa, synthetic construct; identical to SEQ ID NO: 18
  REGION 1..262: note = bTrCP2-263

SEQ ID NO: 207 - protein, 262 aa, synthetic construct
  REGION 1..262: note = bTrCP2-263 variant 7
DPAEAVLQEKALKFMNSSEREDCNNGEPPRKIIPEKNSLRQTYNSCARLCLNQETVCLASTAMKTENCVAKTKLANGTSSMIVPKQRKLSASYEKEKELCVKYFEQWSGSDQVGFVEHLIPQMCHYQHGHINSYLKPMLQRDFITALPARGLDHIAENILSYLDAKSLRAAELVCKEWYRVTSDGMLWKKLIERMVRTDSLWRGLAERRGWGQYLFKNKPPDGYAPPNSFYRALYPKIIQDIETIESNWRCGRHSLQRIHCR

SEQ ID NO: 208 - protein, 262 aa, synthetic construct
  REGION 1..262: note = bTrCP2-263 variant 9
DPAEAVPQEKALKFMNSTEREDCNNGEPPRKIIPEKNSLRQTYNSCARLCLNQETVCLASTAMKTENCVAKTKLANGTSSMIVPKQRKLSASYEKEKELCVKYFEQWSESDQVEFVEHLISQMCHYQHGHINSYLKPMLQRDFITALPARGLDHIAENILSYLDAKSLCAAELVCKEWYRVTSGGMLWKKPIERMVRTDSLWRGLAERRGWGQYLFKNKPPDGNAPPNSFYRALCPKIMQDIETIESNWGCGRHSLQRIHCR

SEQ ID NO: 209 - protein, 262 aa, synthetic construct
  REGION 1..262: note = bTrCP2-263 E1 variant
DPAEAVLQEKALKFLNSSEREDCNNGEPPRKIIAEKDSLRQTYNSCARLCLNQETVCLASTAMKTENCVAKTKLANGTSSMIVPKQRKLSASYGKERELCVKYLEQWSGSDQVGFVEHLIPQVCHYQHGHTNSYLKPMLQRDFITALPARGLDHIAENILSYLDAKSLRAAELVCKEWYRVTSEGMLWKKLIERMVRTDSQWRGLAERRGWGQYLFKNKPPDGYAPPNSFYRALYPKIIQDIETIESNRRCGRHSLQRIHCR

SEQ ID NO: 210 - protein, 262 aa, synthetic construct
  REGION 1..262: note = bTrCP2-263 E2 variant
DPAEAVLQEKALKFMNSSEREDCNNGEPPRKIIPEKNSLRQTYNSSARLCLNQETVCLASTAMKTENCVAKTKLANGTSSMIVPKQRKLSASYEKEKELCVKYFEQWSGSDQVGFVEHLIPQMCHYQHGHINSYLKPMLQRDFITALPARGLDHIAEKILSYLDAKSLRAAELVCKEWYRVTSDGMLWKKLIERMVRTDSRWRGLAERRGWGQYLFKNKPPDGYAPPNSFYRALYPKIIQDIETIESNWRCGRHSLQRIHCR

SEQ ID NO: 211 - protein, 262 aa, synthetic construct
  REGION 1..262: note = bTrCP2-263 E3 variant
DPAEAVLQEKALKFMNSSEREDCNNGEPPRKTIPEKNSLRQTYNSCARLCLNQETVCLASTAMKTENCVAKTKLANGTSSMIVPKQRKLSASYEKEKELCVKYFEQWSGSDQVGFVEHLIPQMCHYQHGHINSYLKPMLQRDFITALPARGLDHIAEKILSYLDAKSLRAAELVCKEWYRVTSDGMLWKKLIERMVRTDSLWRGLAERRGWGQYLFKNKPPDGYAPPNSFYRALYPKIIQEIETIESNRRCGRHSLQRSHCR

SEQ ID NO: 212 - protein, 262 aa, synthetic construct
  REGION 1..262: note = bTrCP2-263 E4 variant
DPAEAVPQEKALKFMNSTEREDCNNGEPPRKIIPEKNSLRQTYNSCARLCLNQETVCLASTAMKTENCVAKTKLANGTSSMIVPKQRKLSASYEKEKELCVKYFEQWSESDQVEFVEHLISQMRHYQHGHINSYLKPMLQRDFIPALPARGLDHIAENILSYLDAKSLCAAVLVCKEWYRVSSGGMLWKKPIERMVRTDSLWGGLAERRGWGQYLFKNKPPDGNAPPNSFYRALCPKIMQDIETIESNWGCGRHSLQRIHCR

SEQ ID NO: 213 - protein, 262 aa, synthetic construct
  REGION 1..262: note = bTrCP2-263 E5 variant
DPAEAVPQVEALKFMNSTEREDCNNGEPPRKIIPEKNSLRQTYNSCARLCLNQETVCLASTAMKTENCVAKTKLANGTSSMIVPKQRKLTASYEKEKELCAKYFEQWSESDQVEFVEHPISQMCHYQHGHINSYLKPMLQRDFITALPARGLDHIAENILSYLDAKSLCAAVLVCKEWYRVTSGGMLWKKPIERMAGTDSLWRGLAERRGWGQYLFKNKPPDGNAPPNSFYRALCPKIMRDIETIESNWGCGRHSLQRIHCR

SEQ ID NO: 214 - protein, 262 aa, synthetic construct
  REGION 1..262: note = bTrCP2-263 E6 variant
DPAEAVPQEKALKFMNSTEREDCNNGGPPRKIIPEKNSLRQTYNSCARLCLNQETVCLASTAMKTENCVAKTKLANGTSSMIVPKQRKLSASYEKERELCVKYFEQWSESDQAEFVEHLISQMCHCQHGHINSYLKPMLQRDSITAPPARGLDHIAENILSYLDAKSLCAVELVCKEWYRVSSGGMLWKKPIERMVRTDSLRRGLAERRGWGQYLFKNKPPDGNAPPNSFYRVLCPKIMRDIETIESNWGCGRHSLQRIHCR

SEQ ID NO: 215 - protein, 175 aa, synthetic construct
  REGION 1..175: note = SKP2 2-176 variant 3
RRRHLQEIPGLSSNVATSFTWGRDSSKTSELLSGMGVSALEKEEPDSENIPQELLSNPGHPESPPRKRLKSKGSDKDFVIVRRPKLNRENFPGVSWDSLPDELLLRIFSRLRLPELLKVSGVCKRWYRLASDESLWKTLDLTGKNLHPDVTGRLLSQGVVAFRCPRSFMDQPLAG

SEQ ID NO: 216 - protein, 175 aa, synthetic construct
  REGION 1..175: note = SKP2 2-176 variant 15
HRKHLQEIPDPSSNVATSFTWGWDSSKTSELPSGMGVSALEKEEPDSENIPQELLSNLGHPESPPRKRLKSKGSDKGFVIVRRPKLNRENFPGVSWVSLPDELLLGIFSCLCLPELLKVSGVCKRWCRLASDEPLWQTLDLTGKNLRPDVTGRLLSQGVIAFRCPRSFMDQPLAE

SEQ ID NO: 217 - protein, 175 aa, synthetic construct
  REGION 1..175: note = SKP2 2-176 E1 variant
RRRHLQEIPGLSSNVATSFTWGRDSSKTSELLSGMGVSALEKEEPDSENIPQELLSNPGHPESPPRKRLKSKGSDKDFVIVRRPKLNRENFPGVSWDSLPDELLLRIFSRLRLPELLKVSGVSKRWYRLASDESLWKSLDLTGKNLHPDVTGRLLSQGVVAFRCPRSFMDQPLAG

SEQ ID NO: 218 - protein, 175 aa, synthetic construct
  REGION 1..175: note = SKP2 2-176 E2 variant
RRRHLQEIPGLSSNVATSFTWGRDSSKTSELLSGMGVSALEKEEPDSENIPQELLSNPGHPESPPRKRLKSKGSDKDFVIVRRPKLNRENFPGVSWDSLPDELLLRIFSRLRLPELLKVSGVSKRWCRLASDESLWKTLDLTGKNLHPDVTGRLLSQGVAAFRCPRSFMDQPLAG

SEQ ID NO: 219 - protein, 175 aa, synthetic construct
  REGION 1..175: note = SKP2 2-176 E4 variant
HRKHLQEIPDPSSNVATSFTWGWDSSKTSELPSGMGVSALEKEEPDSENIPQELLSNLGHPESPPRKRLKSKGSDKGFVIVRRPKLNRENFPGVSWVSLPDELLLGIFSCPCLPELLKVSGVCKRWCRLASDEPLWQTLDLTGKNLRPDVTGRLRSQGVIAFRCPRSFMDQPLAE

SEQ ID NO: 220 - protein, 175 aa, synthetic construct
  REGION 1..175: note = SKP2 2-176 E 5 variant
HRKHLQEIPDPSSNVATSFTWGWDSSKTSELPSGMGVSALEKKEPDSENIPQELLSNLGHPESPPRKRLKSKGSDKGFVIVRRPKLNRENFPGVSWVSLPDELLLGIFSCPCLPELLKVSGVCKRWCRLASDEPLRQTLDLTGKNLRPDVTGRLLSQGVIAFRCPRSFMDQPLAE

SEQ ID NO: 221 - protein, 175 aa, synthetic construct
  REGION 1..175: note = SKP2 2-176_E6
HRKHLQEIPDPSSNVATGFTWGWDSSKASELPSGMGVSALEKEEPDSENIPQELLSNLGHPESPPRKRLKSKGSDKGFVIVRRPKLNRENFPGVSWVSLPNELLLGIFSCRCLPELLKVSGVCKRWCRQASEEPLWQTLDLTGKNLRPDVTGRLQSQGVIAFRCPRSFMDQPLAE

SEQ ID NO: 222 - DNA, 786 bp, synthetic construct; identical to SEQ ID NO: 114
  source 1..786: mol_type = other DNA
  misc_feature 1..786: note = bTrCP2-263

SEQ ID NO: 223 - DNA, 786 bp, synthetic construct
  source 1..786: mol_type = other DNA
  misc_feature 1..786: note = bTrCP2-263 variant 7
gacccggccgaggcggtgctgcaagagaaggcactcaagtttatgaactcctcagagagagaagactgtaataatggcgaaccccctaggaagataataccagagaagaactcacttagacagacatacaacagctgtgccagactctgcttaaaccaagaaacagtatgtttagcaagcactgctatgaagactgagaattgtgtggccaaaacaaaacttgccaatggcacttccagtatgattgtgcccaagcaacggaaactctcagcaagctatgaaaaggaaaaggaactgtgtgtcaaatactttgagcagtggtcagggtcagatcaagtgggatttgtggaacatcttataccccaaatgtgtcattaccaacatgggcacataaactcgtatcttaaacctatgttgcagagagacttcataactgctctgccagctcggggattggatcatattgctgagaacattctgtcatacctggatgccaaatcactacgtgctgctgaacttgtgtgcaaggaatggtaccgagtgacctctgatggcatgctgtggaagaagcttatcgagagaatggtcaggacagattctctgtggagaggcctggcagaacgaagaggatggggacagtatttattcaaaaacaaacctcctgacgggtacgctcctcccaactctttttatagagcactttatcctaaaattatacaagacattgagacaatagaatctaattggagatgtggaagacatagtttacagaggattcactgccga

SEQ ID NO: 224 - DNA, 786 bp, synthetic construct
  source 1..786: mol_type = other DNA
  misc_feature 1..786: note = bTrCP2-263 variant 9
gacccggccgaggcggtgccgcaagagaaggcactcaagtttatgaactccacagagagagaagactgtaataatggcgaaccccctaggaagataataccagagaagaactcacttagacagacatacaacagctgtgccagactctgcttaaaccaagaaacagtatgtttagcaagcactgctatgaagactgagaattgtgtggccaaaacaaaacttgccaatggcacttccagtatgattgtgcccaagcaacggaaactctcagcaagctatgaaaaggaaaaggaactgtgtgtcaaatactttgagcagtggtcagagtcagatcaagtggaatttgtggaacatcttatatcccaaatgtgtcattaccaacatgggcacataaactcgtatcttaaacctatgttgcagagagatttcataactgctctgccagctcggggattggatcatattgctgagaacattctgtcatacctggatgccaaatcactatgtgctgctgaacttgtgtgcaaggaatggtaccgagtgacctctggtggcatgctgtggaagaagcctatcgagagaatggtcaggacagattctctgtggagaggcctggcagaacgaagaggatggggacagtatttattcaaaaacaaacctcctgacgggaatgctcctcccaactctttttatagagcactttgtcctaaaattatgcaagacattgagacaatagaatctaattggggatgtggaagacatagtttacagaggattcactgccga

SEQ ID NO: 225 - DNA, 786 bp, synthetic construct
  source 1..786: mol_type = other DNA
  misc_feature 1..786: note = bTrCP2-263 E1 variant
gacccggccgaggcggtgctgcaagagaaggcactcaagtttttgaactcctcagagagagaagactgtaataatggcgaaccccctaggaagataatagcagagaaggactcacttagacagacatacaacagctgtgccagactctgcttaaaccaagaaacagtatgtttagcaagcactgctatgaagactgagaattgtgtggccaaaacaaaacttgccaatggcacttccagtatgattgtgcccaagcaacggaaactctcagcaagctatggaaaggaaagggaactgtgtgtcaaataccttgagcagtggtcagggtcagaccaagtgggatttgtggaacatcttataccccaagtgtgtcattaccaacatgggcacacaaactcgtatcttaaacctatgttgcagagagacttcataactgctctgccagctcggggattggatcatattgctgagaacattctgtcatacctggatgccaaatcactacgtgctgctgaacttgtgtgcaaggaatggtaccgagtgacctctgaaggcatgctgtggaagaagcttatcgagagaatggtcaggacagattctcagtggagaggcctggcagaacgaagaggatggggacagtatttattcaaaaacaaacctcctgacgggtacgctcctcccaactctttttatagagcactttatcctaaaattatacaagacattgagacaatagaatctaatcggagatgtggaagacatagtttacagaggattcactgccga

SEQ ID NO: 226 - DNA, 786 bp, synthetic construct
  source 1..786: mol_type = other DNA
  misc_feature 1..786: note = bTrCP2-263 E2 variant
gacccggccgaggcggtgctgcaggagaaggcactcaagtttatgaactcctcagagagagaagactgtaataatggcgaaccccctaggaagataataccagagaagaactcacttagacagacatacaacagcagtgccagactctgcttaaaccaagaaacagtatgtttagcaagcactgctatgaagactgagaattgtgtggccaaaacaaaacttgccaatggcacttccagtatgattgtgcccaagcaacggaaactctcagcaagctatgaaaaggaaaaggaactgtgtgtcaaatactttgagcagtggtcagggtcagaccaagtgggatttgtggaacatcttataccccaaatgtgtcattaccaacatgggcacataaactcgtatcttaaacctatgttgcagagagacttcataactgctctgccagctcggggattggatcatattgctgagaaaattctgtcatacctggatgccaaatcactacgtgctgctgaacttgtgtgcaaggaatggtaccgagtgacctctgatggcatgctgtggaagaagcttatcgagagaatggtcaggacagattctcggtggagaggcctggcagaacgaagaggatggggacagtatttattcaaaaacaaacctcctgacgggtacgctcctcccaactctttttatagagcactttatcctaaaattatacaagacattgagacaatagaatctaattggagatgtggaagacatagtttacagaggattcactgccga

SEQ ID NO: 227 - DNA, 786 bp, synthetic construct
  source 1..786: mol_type = other DNA
  misc_feature 1..786: note = bTrCP2-263 E3 variant
gacccggccgaggcggtgctgcaagagaaggcactcaagtttatgaactcctcagagagagaagactgtaataatggcgaaccccctaggaagacaataccagagaagaactcactcagacagacatacaacagctgtgccagactctgcttaaaccaagaaacagtatgtttagcaagcactgctatgaagactgagaattgtgtggccaaaacaaaacttgccaatggcacttccagtatgattgtgcccaagcaacggaaactctcagcaagctatgaaaaggaaaaggaactgtgtgtcaaatactttgagcagtggtcagggtcagaccaagtgggatttgtggaacatcttataccccaaatgtgtcattaccaacatgggcacataaactcgtatcttaaacctatgttgcagagagacttcataactgctctgccagctcggggattggatcatattgctgagaaaattctgtcatacctggatgccaaatcactacgtgctgctgaacttgtgtgcaaggaatggtaccgagtgacctctgatggcatgctgtggaagaagcttatcgagagaatggtcaggacagattctctgtggagaggcctggcagaacgaagaggatggggtcagtatttattcaaaaacaaacctcctgacgggtacgctcctcccaactctttttatagagcactttatcctaaaattatacaagagattgagacaatagaatctaatcggagatgtggaagacatagtttacagaggagtcactgccga

SEQ ID NO: 228 - DNA, 786 bp, synthetic construct
  source 1..786: mol_type = other DNA
  misc_feature 1..786: note = bTrCP2-263 E4 variant
gacccggccgaggcggtgccgcaagagaaggcactcaagtttatgaactccacagagagagaagactgtaataatggtgaaccccctaggaagataataccagagaagaactcacttagacagacatacaacagctgtgccagactctgcttaaaccaagaaacagtatgtttagcaagcactgctatgaagactgagaattgtgtggccaaaacaaaacttgccaatggcacttccagtatgattgtgcccaagcaacggaaactctcagcaagctatgaaaaggaaaaggaactgtgtgtcaaatactttgagcagtggtcagagtcagatcaagtggaatttgtggaacatcttatatcccaaatgcgtcattaccaacatgggcacataaactcgtatcttaaacctatgttgcagagagatttcatacctgctctgccagctcggggattggatcatattgctgagaacattctgtcatacctggatgccaaatctctatgtgctgctgtacttgtgtgcaaggagtggtaccgagtgtcctctggtggcatgctgtggaagaagcctatcgagagaatggtcaggacagattctctgtggggaggcctggcagaacgaagaggatggggacagtatttattcaaaaacaaacctcctgacgggaatgctcctcccaactctttttatagagcactttgtcctaaaattatgcaagacattgagacaatagaatctaattggggatgtggaagacacagtttacagaggattcactgccga

SEQ ID NO: 229 - DNA, 786 bp, synthetic construct
  source 1..786: mol_type = other DNA
  misc_feature 1..786: note = bTrCP2-263 E5 variant
gacccggccgaggcggtgccgcaagtggaggcactcaagtttatgaactccacagagagagaagactgtaataatggtgaaccccctaggaagataataccagagaagaactcacttagacagacatacaacagctgtgccagactctgcttaaaccaagaaacagtatgtttagcgagcactgctatgaagactgagaattgtgtggccaaaacaaaacttgccaatggcacttccagtatgattgtgcccaagcaacggaaactcacagcaagctatgaaaaggaaaaggaactgtgtgccaaatactttgagcagtggtcagagtcagatcaagtggaatttgtggaacatcctatatcccaaatgtgtcattaccaacatgggcacataaactcgtatcttaaacctatgttgcagagagatttcataactgctctgccagctcggggattggatcatattgctgagaacattctgtcatacctggatgccaaatcactatgtgctgctgtacttgtgtgcaaggagtggtaccgagtgacctctggtggcatgctgtggaagaagcctatcgagagaatggccgggacagattctctgtggagaggcctggcagaacgaagaggatggggacagtatttattcaaaaacaaacctcctgacgggaatgctcctcccaactctttttatagagcactttgtcctaaaattatgcgagacattgagacaatagaatctaattggggatgtggaagacacagtttacagaggattcactgccga

SEQ ID NO: 230 - DNA, 822 bp, synthetic construct
  source 1..822: mol_type = other DNA
  misc_feature 1..587: note = bTrCP_E6
gacccggccgaggcggtgccgcaagagaaggcactcaagtttatgaactccacagagagagaagactgtaataatggtggaccccctaggaagataataccagagaagaactcacttagacagacatacaacagctgtgccagactctgcttaaaccaagaaacagtatgtttagcaagcactgctatgaagactgagaattgtgtggccaaaacaaaacttgccaatggcacttccagtatgattgtgcccaagcaacggaaactctcagcaagctatgaaaaggaaagggaactgtgtgtcaaatactttgagcagtggtcagagtcagatcaagcggaatttgtggaacatcttatatcccaaatgtgtcattgccaacatgggcacataaactcgtatcttaaacctatgttgcagagagattccataactgctccgccagctcggggattggatcatattgctgagaacattctgtcatacctggatgccaaatcactatgtgctgttgaacttgtgtgcaaggagtggtaccgagtgtcctctggtggcatgctgtggaagaagcctatcgagagaatggtcaggacagattctctgcggagaggcctggcagaacgaagaggatggggacagtatttattcaaaaacaaacctcctgacgggaatgctcctcccaactctttttatagagtactttgtcctaaaattatgcgagacattgagacaatagaatctaattggggatgtggaagacacagtttacagaggattcactgccgaggatccgaacaaaagcttatctccgaagaagacttg

SEQ ID NO: 231 - DNA, 525 bp, synthetic construct
  source 1..525: mol_type = other DNA
  misc_feature 1..525: note = SKP2 2-176 variant 3
cgcaggaggcacctccaggagattccaggcctgagtagcaacgttgccaccagcttcacgtggggacgggattccagcaagacttctgaactgctgtcaggcatgggggtctccgccctggagaaagaggagcccgacagtgagaacatcccccaggaactgctctcaaacccgggccacccggagagccccccacggaaacggctgaagagcaaagggagtgacaaagactttgtgattgtccgcaggcctaagctaaaccgagagaactttccaggcgtttcatgggactcccttccggatgagctgctcttgagaatcttttcccgtctgcgcctccctgagctgctaaaggtctctggtgtttgtaagaggtggtatcgcctagcgtctgatgagtctctatggaagaccttagacctcacaggtaaaaatctgcacccggatgtgactggtcggttgctgtcccaaggggtggttgccttccgctgcccacgatcatttatggaccaaccattggctgga

SEQ ID NO: 232 - DNA, 525 bp, synthetic construct
  source 1..525: mol_type = other DNA
  misc_feature 1..525: note = SKP2 2-176 variant 15
cacaggaagcacctccaggagattccagacccgagtagcaacgttgccaccagcttcacgtggggatgggattccagcaagacttctgaactgccgtcaggcatgggggtctccgccctggagaaagaggagcccgacagtgagaatatcccccaggaactgctctcaaacctgggccacccggagagccccccacggaaacggctgaagagcaaagggagtgacaaaggctttgtgattgtccgcaggcctaagctaaatcgagagaactttccaggtgtttcgtgggtctcccttccggatgagctgctcttgggaatcttttcctgtctgtgcctccctgagctgctaaaggtctctggtgtttgcaagaggtggtgtcgcctagcgtctgatgagcctctatggcagaccttagacctcacaggtaaaaatctgcgcccggatgtgactggtcggttgctgtctcaaggggtgattgccttccgctgccctcgatcatttatggaccaaccattggccgaa

SEQ ID NO: 233 - DNA, 525 bp, synthetic construct
  source 1..525: mol_type = other DNA
  misc_feature 1..525: note = SKP2 2-176 E1 variant
cgcaggaggcacctccaggagattccaggcctgagtagcaacgttgccaccagcttcacgtggggacgggattccagcaagacttctgaactgctgtcaggcatgggggtctccgccctggagaaagaggagcccgacagtgagaacatcccccaggaactgctctcaaacccgggccacccggagagccccccacggaaacggctgaagagcaaagggagtgacaaagactttgtgattgtccgcaggcctaagctaaaccgagagaactttccaggcgtttcatgggactcccttccggatgagctgctcttgagaatcttttcccgtctgcgcctccctgagctgctaaaggtctctggtgttagtaagaggtggtatcgcctagcgtctgatgagtctctatggaagagcttagacctcacaggtaaaaatctgcacccggatgtgactggtcggttgctgtcccaaggggtggttgccttccgctgcccacgatcatttatggaccaaccattggctgga

SEQ ID NO: 234 - DNA, 525 bp, synthetic construct
  source 1..525: mol_type = other DNA
  misc_feature 1..525: note = SKP2 2-176 E2 variant
cgcaggaggcacctccaggagattccaggcctgagtagcaacgttgccaccagcttcacgtggggacgggattccagcaagacttctgaactgctgtcaggcatgggggtctccgccctggagaaagaggagcccgacagtgagaacatcccccaggaactgctctcaaacccgggccacccggagagccccccacggaaacggctgaagagcaaagggagtgacaaagactttgtgattgtccgcaggcctaagctaaaccgagagaactttccaggcgtttcatgggactcccttccggatgagctgctcttgagaatcttttcccgtctgcgcctccctgagctgctaaaggtctctggtgttagtaagaggtggtgtcgcctagcgtctgatgagtctctatggaagaccttagacctcacaggtaaaaatctgcacccggatgtgactggtcggttgctgtcccaaggggtggctgccttccgctgcccacgatcatttatggaccaaccattggctgga

SEQ ID NO: 235 - DNA, 525 bp, synthetic construct
  source 1..525: mol_type = other DNA
  misc_feature 1..525: note = SKP2 2-176 E4 variant
cacaggaagcacctccaggagattccagacccgagtagcaacgttgccaccagcttcacgtggggatgggattccagcaagacttctgaactgccgtcaggcatgggggtctccgccctggagaaagaggagcccgacagtgagaatatcccccaggaactgctctcaaacctgggccacccggagagccccccacggaaacggctgaagagcaaagggagtgacaaaggctttgtgattgtccgcaggcctaagctaaatcgagagaactttccaggtgtttcgtgggtctcccttccggatgagctgctcttgggaatcttttcctgtccgtgcctccctgagctgctaaaggtctctggtgtttgcaagaggtggtgtcgcctagcgtctgatgagcctctatggcagaccttagacctcacaggtaaaaatctgcgcccggatgtgactggtcggttgcggtctcaaggggtgattgccttccgctgccctcggtcatttatggaccaaccattggccgaa

SEQ ID NO: 236 - DNA, 525 bp, synthetic construct
  source 1..525: mol_type = other DNA
  misc_feature 1..525: note = SKP2 2-176 E 5variant
cacaggaagcacctccaggagattccagacccgagtagcaacgttgccaccagcttcacgtggggatgggattccagcaagacttctgaactgccgtcaggcatgggggtctccgccctggagaaaaaggagcccgacagtgagaatatcccccaggaactgctctcaaacctgggccacccggagagccccccacggaaacggctgaagagcaaagggagtgacaaaggctttgtgattgtccgcaggcctaagctaaatcgtgagaactttccaggtgtttcgtgggtctcccttccggatgagctgctcttgggaatcttttcctgtccgtgcctccctgagctgctaaaggtctctggtgtttgcaagaggtggtgtcgcctagcgtctgatgagcctctaaggcagaccttagacctcacaggtaaaaatctgcgcccggatgtgactggtcggttgctgtctcaaggggtgattgccttccgctgccctcgatcatttatggaccaaccattggccgaa

SEQ ID NO: 237 - DNA, 525 bp, synthetic construct
  source 1..525: mol_type = other DNA
  misc_feature 1..525: note = SKP2 2-176 E6 variant
cacaggaagcacctccaggagattccagacccgagtagcaacgttgccaccggcttcacgtggggatgggattccagcaaggcttctgaactgccgtcaggcatgggggtctccgccctggagaaagaggagcccgacagtgagaatatcccccaggaactgctctcaaacctgggccacccggagagccccccacggaaacggctgaagagcaaagggagtgacaaaggctttgtgattgtccgcaggcctaagctaaatcgagagaactttccaggtgtttcgtgggtctcccttccgaatgagctgctcttgggaatcttttcctgtcggtgcctccctgagctgctaaaggtctctggtgtttgtaagaggtggtgtcgccaagcgtctgaagagcctctatggcagaccttagacctcacaggtaaaaatctgcgcccggatgtgactggtcggttgcagtctcaaggggtgattgccttccgctgccctcgatcatttatggaccaaccattggctgaa

SEQ ID NO: 238 - protein, 15 aa, synthetic construct
  REGION 1..15: note = linker
GGGGSGGGGSGGGGS

SEQ ID NO: 239 - DNA, 45 bp, synthetic construct
  source 1..45: mol_type = other DNA
  misc_feature 1..45: note = linker
ggtggaggcggttcaggcggaggtggctctggcggtggcggatcg

SEQ ID NO: 240 - protein, 299 aa, synthetic construct
  REGION 1..299: note = pNLF1-N-S14
MVFTLEDFVGDWRQTAGYNLDQVLEQGGVSSLFQNLGVSVTPIQRIVLSGENGLKIDIHVIIPYEGLSGDQMGQIEKIFKVVYPVDDHHFKVILHYGTLVIDGVTPNMIDYFGRPYEGIAVFDGKKITVTGTLWNGNKIIDERLINPDGSLLFRVTINGVTGWRLCERILAGSSGAIASEFQVKLEESGGGSVQTGGSLRLTCAASGSIFSMNRMGWFRQAPGKERELVAVIDSKRNKTHYADSVKGRFTISRDNAKNTVDLQMNSLKPEDTAIYYCTAWTGRPPRGYWGQGTQVTVSS

SEQ ID NO: 241 - protein, 299 aa, synthetic construct
  REGION 1..299: note = pNLF1-N-2E8
MVFTLEDFVGDWRQTAGYNLDQVLEQGGVSSLFQNLGVSVTPIQRIVLSGENGLKIDIHVIIPYEGLSGDQMGQIEKIFKVVYPVDDHHFKVILHYGTLVIDGVTPNMIDYFGRPYEGIAVFDGKKITVTGTLWNGNKIIDERLINPDGSLLFRVTINGVTGWRLCERILAGSSGAIASEFEVQLVESGGGLVQPGGSLRLSCAASGFTLDYYGMGWFRQAPGKEREFVAAISRSGGSTVYADSVKGRFTISADNSKNTAYLQMNSLKPEDTAVYYCAREVVRGGINYWGQGTLVTVSS

SEQ ID NO: 242 - protein, 307 aa, synthetic construct
  REGION 1..307: note = pNLF1-N-3F11
MVFTLEDFVGDWRQTAGYNLDQVLEQGGVSSLFQNLGVSVTPIQRIVLSGENGLKIDIHVIIPYEGLSGDQMGQIEKIFKVVYPVDDHHFKVILHYGTLVIDGVTPNMIDYFGRPYEGIAVFDGKKITVTGTLWNGNKIIDERLINPDGSLLFRVTINGVTGWRLCERILAGSSGAIASEFDVQLVESGGGLVQPGGSLRLSCATSGFTFSSSTMSWVRQVPGAGPEWVAVDNPGGKKNYIDSVAGRFTIARDNDANSLSLVMNGLRPEDTARYFCARVLSFKIYEGDKWALEWDYRGPGTQVTVSS

SEQ ID NO: 243 - protein, 307 aa, synthetic construct
  REGION 1..307: note = pNLF1-N-3A2
MVFTLEDFVGDWRQTAGYNLDQVLEQGGVSSLFQNLGVSVTPIQRIVLSGENGLKIDIHVIIPYEGLSGDQMGQIEKIFKVVYPVDDHHFKVILHYGTLVIDGVTPNMIDYFGRPYEGIAVFDGKKITVTGTLWNGNKIIDERLINPDGSLLFRVTINGVTGWRLCERILAGSSGAIASEFEVQLVESGGEQVQPGSSLKLSCSVSGLMISGHAMSWVRQVPGAGPEWVAVDNPGGKKNYIDSVAGRFTIARDNDANSLSLVMNGLRPEDTARYFCARVLSFKIYEGDKWALEWDYRGPGTQVTVSS

SEQ ID NO: 244 - protein, 307 aa, synthetic construct
  REGION 1..307: note = pNLF1-N-3H9
MVFTLEDFVGDWRQTAGYNLDQVLEQGGVSSLFQNLGVSVTPIQRIVLSGENGLKIDIHVIIPYEGLSGDQMGQIEKIFKVVYPVDDHHFKVILHYGTLVIDGVTPNMIDYFGRPYEGIAVFDGKKITVTGTLWNGNKIIDERLINPDGSLLFRVTINGVTGWRLCERILAGSSGAIASEFQVQLVESGGEQVQPGSSLKLSCSVSGLMISGHAMSWVRQVPGAGPEWVAVDNPGGKKNYIDSVAGRFTIARDNDANSLSLVMNGLRPEDTARYFCARVLSFKIYGGDKWALEWDYRGPGTQVTVSS

SEQ ID NO: 245 - DNA, 897 bp, synthetic construct
  source 1..897: mol_type = other DNA
  misc_feature 1..897: note = pNLF1-N-S14
atggtcttcacactcgaagatttcgttggggactggcgacagacagccggctacaacctggaccaagtccttgaacagggaggtgtgtccagtttgtttcagaatctcggggtgtccgtaactccgatccaaaggattgtcctgagcggtgaaaatgggctgaagatcgacatccatgtcatcatcccgtatgaaggtctgagcggcgaccaaatgggccagatcgaaaaaatttttaaggtggtgtaccctgtggatgatcatcactttaaggtgatcctgcactatggcacactggtaatcgacggggttacgccgaacatgatcgactatttcggacggccgtatgaaggcatcgccgtgttcgacggcaaaaagatcactgtaacagggaccctgtggaacggcaacaaaattatcgacgagcgcctgatcaaccccgacggctccctgctgttccgagtaaccatcaacggagtgaccggctggcggctgtgcgaacgcattctggcgggctcgagcggcgcgatcgcttccgaattccaggtgaagctggaggagagcggcggcggcagcgtgcagaccggcggcagcctgaggctgacctgcgccgccagcggcagcatcttcagcatgaacaggatgggctggttcaggcaggcccccggcaaggagagggagctggtggccgtgatcgacagcaagaggaacaagacccactacgccgacagcgtgaagggcaggttcaccatcagcagggacaacgccaagaacaccgtggacctccagatgaacagcctgaagcccgaggacaccgccatctactactgcaccgcctggaccggcaggccccccaggggctactggggccagggcacccaggtgaccgtgagcagc

SEQ ID NO: 246 - DNA, 897 bp, synthetic construct
  source 1..897: mol_type = other DNA
  misc_feature 1..897: note = pNLF1-N-2E8
atggtcttcacactcgaagatttcgttggggactggcgacagacagccggctacaacctggaccaagtccttgaacagggaggtgtgtccagtttgtttcagaatctcggggtgtccgtaactccgatccaaaggattgtcctgagcggtgaaaatgggctgaagatcgacatccatgtcatcatcccgtatgaaggtctgagcggcgaccaaatgggccagatcgaaaaaatttttaaggtggtgtaccctgtggatgatcatcactttaaggtgatcctgcactatggcacactggtaatcgacggggttacgccgaacatgatcgactatttcggacggccgtatgaaggcatcgccgtgttcgacggcaaaaagatcactgtaacagggaccctgtggaacggcaacaaaattatcgacgagcgcctgatcaaccccgacggctccctgctgttccgagtaaccatcaacggagtgaccggctggcggctgtgcgaacgcattctggcgggctcgagcggcgcgatcgcttccgaattcgaagtgcagctggtggaaagcggcggcggcctggtgcagccgggcggcagcctgcgcctgagctgcgcggcgagcggctttaccctggattattatggcatgggctggtttcgccaggcgccgggcaaagaacgcgaatttgtggcggcgattagccgcagcggcggcagcaccgtgtatgcggatagcgtgaaaggccgctttaccattagcgcggataacagcaaaaacaccgcgtatctgcagatgaacagcctgaaaccggaagataccgcggtgtattattgtgcacgcgaagttgtacgtggtggtattaattattggggccagggcaccctggtgaccgtgagcagc

SEQ ID NO: 247 - DNA, 921 bp, synthetic construct
  source 1..921: mol_type = other DNA
  misc_feature 1..921: note = pNLF1-N-3F11
atggtcttcacactcgaagatttcgttggggactggcgacagacagccggctacaacctggaccaagtccttgaacagggaggtgtgtccagtttgtttcagaatctcggggtgtccgtaactccgatccaaaggattgtcctgagcggtgaaaatgggctgaagatcgacatccatgtcatcatcccgtatgaaggtctgagcggcgaccaaatgggccagatcgaaaaaatttttaaggtggtgtaccctgtggatgatcatcactttaaggtgatcctgcactatggcacactggtaatcgacggggttacgccgaacatgatcgactatttcggacggccgtatgaaggcatcgccgtgttcgacggcaaaaagatcactgtaacagggaccctgtggaacggcaacaaaattatcgacgagcgcctgatcaaccccgacggctccctgctgttccgagtaaccatcaacggagtgaccggctggcggctgtgcgaacgcattctggcgggctcgagcggcgcgatcgcttccgaattcgacgttcagctcgtcgaaagtggaggtgggttggtacagcccggaggaagcctcagactctcatgtgcaacgagcggcttcacgtttagcagcagtaccatgtcctgggttcgacaggtaccgggtgcaggcccagagtgggtagccgtcgataatcctggcggcaaaaagaactacatcgacagtgttgcaggacggtttaccatagcacgcgacaacgacgctaattccctctcccttgtgatgaatggattgaggccagaagacacagctaggtatttctgtgccagggtacttagcttcaaaatctatgaaggagataagtgggctttggaatgggactatcgcggccctggcacccaggtgaccgtctccagc

SEQ ID NO: 248 - DNA, 921 bp, synthetic construct
  source 1..921: mol_type = other DNA
  misc_feature 1..921: note = pNLF1-N-3A2
atggtcttcacactcgaagatttcgttggggactggcgacagacagccggctacaacctggaccaagtccttgaacagggaggtgtgtccagtttgtttcagaatctcggggtgtccgtaactccgatccaaaggattgtcctgagcggtgaaaatgggctgaagatcgacatccatgtcatcatcccgtatgaaggtctgagcggcgaccaaatgggccagatcgaaaaaatttttaaggtggtgtaccctgtggatgatcatcactttaaggtgatcctgcactatggcacactggtaatcgacggggttacgccgaacatgatcgactatttcggacggccgtatgaaggcatcgccgtgttcgacggcaaaaagatcactgtaacagggaccctgtggaacggcaacaaaattatcgacgagcgcctgatcaaccccgacggctccctgctgttccgagtaaccatcaacggagtgaccggctggcggctgtgcgaacgcattctggcgggctcgagcggcgcgatcgcttccgaattcgaggtgcaattggttgagtcaggaggtgagcaggtccaacctggtagttctttgaaattgagctgttcagtctcaggtctgatgatatcaggccacgcgatgagttgggtcaggcaagtaccgggggccgggcctgagtgggtcgcggtggataatccagggggtaaaaagaactatattgactcagttgctggcagatttacgattgctcgggacaacgatgcaaactctctgagcctcgttatgaacggtctgcggcctgaggacacagccaggtacttctgcgcccgagtattgagctttaagatatacgaaggagataaatgggctctggagtgggactatcgcgggccgggcacacaagtgacggtgtccagc

SEQ ID NO: 249 - DNA, 921 bp, synthetic construct
  source 1..921: mol_type = other DNA
  misc_feature 1..921: map = pNLF1-N-3H9
atggtcttcacactcgaagatttcgttggggactggcgacagacagccggctacaacctggaccaagtccttgaacagggaggtgtgtccagtttgtttcagaatctcggggtgtccgtaactccgatccaaaggattgtcctgagcggtgaaaatgggctgaagatcgacatccatgtcatcatcccgtatgaaggtctgagcggcgaccaaatgggccagatcgaaaaaatttttaaggtggtgtaccctgtggatgatcatcactttaaggtgatcctgcactatggcacactggtaatcgacggggttacgccgaacatgatcgactatttcggacggccgtatgaaggcatcgccgtgttcgacggcaaaaagatcactgtaacagggaccctgtggaacggcaacaaaattatcgacgagcgcctgatcaaccccgacggctccctgctgttccgagtaaccatcaacggagtgaccggctggcggctgtgcgaacgcattctggcgggctcgagcggcgcgatcgcttccgaattccaggtacagcttgtcgagtccggcggcgaacaagtacaaccaggatcttccctgaaattgtcttgctccgtctcaggtcttatgattagcggccacgcgatgtcttgggtaaggcaagtaccaggggcgggacccgaatgggtcgcggtcgataaccctggtggaaagaaaaactacattgactccgttgcggggcggtttacgatagctcgggacaatgatgccaattcactttccctggttatgaacggcctccgaccagaggataccgctcgatacttctgcgccagagtactttcttttaagatttatggtggggataaatgggctcttgaatgggactatcgaggacctggaactcaagttaccgtaagcagc